European Patent Application EP 4 174 175 A1, published May 3, 2023. Title: HYALURONIC ACID-PRODUCING RECOMBINANT CELLS. Applicant: GIVAUDAN SA. The sequence listing filed with the application follows.

SEQUENCE LISTING (108 sequences)

SEQ ID NO: 1 - DNA, 1707 bp, Paramecium bursaria Chlorella virus 1
  "Reencoded nucleic acid sequence of hyaluronan synthase (HASA) originating from Chlorella virus PBCV-1"
  Reencoded nucleic acid sequence of hyaluronan synthase (HASA) originating from Chlorella virus PBCV-1
atgggtaagaacatcattattatggtttcttggtacactattattacatccaatctcatcgcagtgggtggcgcctcactcatactagccccagctattacgggctatgtccttcactggaacattgccctttcaacaatttggggagtgtcggcctacggaattttcgtgtttggtttctttcttgcccaggtattatttagtgaactcaaccggaaaaggctccggaagtggatttccctccgacccaaagggtggaatgatgttaggttggctgtaattattgccggctaccgtgaggacccgtatatgttccaaaagtgtcttgaaagtgtgcgtgactcagactatgggaatgtagctagactaatatgcgttattgacggcgatgaagacgacgacatgaggatggctgcagtgtacaaggctatctataacgacaacatcaagaaacctgagtttgtcctctgtgagagtgacgataaggagggtgagagaatagatagcgatttcagccgtgatatctgcgtgctgcaaccgcatcgcggaaagcgtgaatgtttgtacacagggttccaattggcaaagatggacccctcagttaatgccgtcgtcctaatcgacagtgacactgtgttagaaaaggacgcgattctcgaagtagtatacccgctggcatgcgatccagaaatacaggctgtagcaggcgaatgcaaaatatggaatactgacacactgttgagtttgctggtagcctggcgatattacagcgcattttgcgtagagcgtagcgcccaatcattcttcaggacagtacaatgcgtcggaggacctctcggcgcctacaagattgatataattaaggaaatcaaggacccatggatcagccaacgtttccttggccaaaagtgcacatacggcgacgatagacgactcactaatgaaatactaatgaggggtaagaaagtagttttcaccccattcgctgttggctggtccgacagcccgacgaacgtcttccgttacattgtacagcaaacacggtggtccaagtcgtggtgtagggagatatggtatacactgtttgcagcatggaagcatggactttcgggcatttggctcgcattcgagtgcttataccagattacttatttcttcctggtgatttacctattctcccgtttggctgttgaggctgacccacgggcgcaaacggccaccgtcattgtttcgaccacagttgcgcttattaagtgcggttactttagcttcagagctaaagacattagggccttctatttcgtcctctacacgttcgtttacttcttctgcatgattccggcacgaataactgcgatgatgaccctgtgggacataggttggggaaccaggggaggaaatgagaagccttccgtaggcaccagagttgctttgtgggccaagcaatatttgattgcttacatgtggtgggccgctgtcgtcggtgctggcgtgtactccatcgttcataattggatgtttgactggaattcactttcctacaggttcgcactggtaggcatctgttcgtatatagttttcattgtaatagtgctggtagtctactttacaggaaagatcacgacctggaacttcacgaagctacagaaagaattgatcgaggaccgcgtactgtacgacgcaacgaccaatgcccagtcggtataa

SEQ ID NO: 2 - DNA, 1707 bp, Paramecium bursaria Chlorella virus 1
  "Reencoded nucleic acid sequence of hyaluronan synthase (HASA) originating from Chlorella virus PBCV-1"
  Reencoded nucleic acid sequence of hyaluronan synthase (HASA) originating from Chlorella virus PBCV-1
atgggcaagaatattattatcatggtcagttggtataccattattacatcaaacctaattgctgtcggtggagcctcactaatcttagctcccgcgattacgggttatgtgcttcattggaatattgctttatccactatttggggtgttagcgcttacggcatctttgtgttcggtttcttcttggctcaggtgttattctctgagctaaacagaaagagactcagaaagtggatttcgctgcggccgaagggatggaacgatgttcggttagcggtgatcattgccggttatcgtgaagatccttatatgtttcagaagtgtttggaatctgttcgagactcagactacggtaacgttgctaggctgatctgcgtaatcgatggagacgaagatgacgatatgagaatggccgcggtttataaagccatctataacgataacattaagaagccagagtttgttttatgcgaatcggatgacaaggagggtgagaggattgattctgacttctcgcgtgacatctgtgtcctgcagccccacaggggaaagcgagagtgcctctatacaggattccaattagctaaaatggacccaagcgttaatgctgtcgtccttatcgatagcgacacggtgttggaaaaggacgcaatattggaagtagtctatccactcgcttgtgatccagagatccaggccgtggctggcgagtgcaagatttggaatacagatacgcttctgtcattactggtggcgtggcgttattattcagcattctgtgtggagaggagcgcacaatcgttctttcggactgtacaatgcgtaggcggtccactaggagcatataaaattgacataatcaaagagataaaagatccttggatttcgcagagattcctcggtcaaaagtgtacctatggggacgacaggcggttgactaacgagattctaatgagaggtaagaaggtggtgttcactccttttgcggtaggttggagcgattcgcccacaaatgtattcagatacattgttcaacaaacaaggtggtcgaaatcgtggtgccgagaaatatggtacacgttgttcgccgcatggaaacacggcttgtcgggtatatggctcgctttcgagtgcctttatcagatcacttacttcttcctggttatttacttgttttcaagactggcagtggaagctgatccaagggctcagactgctactgtcatcgtttcaacaacagtggcgctaataaagtgtggttacttcagctttcgcgcgaaggacataagagcgttttactttgttctttatacctttgtatatttcttctgtatgatcccggcccggataacagctatgatgacattatgggacattggttggggcaccaggggtgggaatgagaagccgtccgtaggaacgagagtagcgctgtgggccaagcagtatcttatcgcatacatgtggtgggcagctgtcgtcggggcaggtgtatacagcatagtacataactggatgtttgactggaactcactctcatatcgattcgcattggtcgggatctgctcttacatcgtgtttattgttatagtcttagtagtatatttcactggaaagataacaacatggaatttcactaagcttcaaaaggaattgattgaagacagggtgctctacgatgcgacaactaatgcacaaagcgtataa

SEQ ID NO: 3 - DNA, 2919 bp, Pasteurella multocida
  "Reencoded nucleic acid sequence of hyaluronan synthase (HASA) originating from Pasteurella multocida"
  Reencoded nucleic acid sequence of hyaluronan synthase (HASA) originating from Pasteurella multocida
atgaacaccctttcccaggcaattaaggcttataatagtaatgattatcaactagccctcaagctgttcgaaaagtcggcagaaatctacggcagaaagatagttgagttccaaattacgaagtgcaaggagaaactttctgcgcacccatccgttaacagtgcgcatctctcggttaacaaagaagagaaggtgaatgtttgcgacagtccattagacatagccactcaattattgttatcgaatgtgaaaaaactcgtccttagtgatagcgagaaaaatacactaaagaataaatggaagttgttgactgaaaagaagtctgagaacgcagaggtccgggccgtagctttagttcccaaggactttccgaaagatttagtgcttgcgccgttaccagaccatgtgaacgattttacgtggtataagaagcggaagaaacgcctaggaatcaaaccagaacaccaacacgttggcctctccattattgtgacaacgttcaaccgtcctgccatcctcagcatcaccctggcttgcctcgtcaatcaaaagacccattatccttttgaggtgatcgtgaccgacgatggttctcaagaggatttatcgcctataatccgtcaatatgagaacaagctagacatccgttatgttcggcaaaaggacaacggttttcaggcatcggccgcacgtaatatgggcctacgtctagccaaatatgacttcattgggctccttgattgtgatatggctcccaaccctttgtgggtacactcatacgttgcggaactattagaggacgatgatttgaccataataggccccaggaagtacattgacacgcaacacatagatcccaaggatttccttaataacgcctctctgttagagtcgttgccagaggttaagaccaataattccgtcgcggctaagggcgaggggaccgtatctttagactggcgtttggaacaatttgagaagaccgagaacttgaggctatccgatagccctttccgattcttcgcagctgggaatgtggctttcgccaagaagtggcttaacaagtcaggattcttcgacgaggaattcaatcactggggaggtgaagatgtagagttcggttatcgtctgtttcggtacggttcgttcttcaaaactatagacggcatcatggcctatcatcaggaaccgccaggtaaagaaaacgaaactgacagagaagcgggcaagaacattaccctcgatataatgagggagaaggtgccttacatctaccgtaaactcctgcctatagaagacagtcatatcaaccgagtaccattggtatcaatttacatcccggcctacaactgtgctaactatattcaaagatgtgttgattcagctttgaatcaaacggtagttgatctcgaagtgtgcatttgcaacgacggtagtactgacaacacgctggaagttattaacaagctgtatggtaataatccgcgtgtgcgtataatgtctaaacccaatggcggcattgcgagtgcatccaacgcagcggtcagcttcgcaaagggttattacataggacagttggacagcgacgattacttagaacccgacgcagtggagttatgtctcaaggaatttcttaaggataagacccttgcgtgcgtttacaccactaatcgtaacgtcaacccagatggctctttaatagccaatggctataactggccagagttcagtcgtgagaagttgactacggccatgattgctcatcacttccggatgtttaccattcgtgcttggcatctgacggatgggttcaatgagaagattgagaacgctgttgactacgacatgtttctcaagctcagtgaagttggtaaatttaagcatctgaacaaaatatgttataatcgggtgttacacggcgataacacctcaatcaagaagcttggcatacaaaagaagaatcatttcgtagttgtcaatcagtctctaaaccgccaaggtataacttattataactacgatgaatttgatgatctcgatgagagtcggaaatacattttcaacaagactgcagagtatcaagaagagatagatattcttaaagatattaagatcattcagaacaaagacgccaaaatagctgtctccattttctatccgaacactctaaacgggttggtgaagaagctaaataatattatagagtataataagaatatcttcgttattgtacttcatgtcgataagaatcacttaaccccagacatcaagaaggagatattagccttctaccataagcatcaggtgaacatcttattgaacaatgacatctcctactatacatcaaatcgtctgattaagacagaagcccatttgagtaacattaacaagctaagtcaattaaatcttaactgcgaatacattatattcgacaatcacgattccttatttgtgaagaacgattcctatgcatacatgaagaagtatgatgttggaatgaacttctctgcattgactcatgattggattgaaaagataaacgctcacccgccatttaagaagctgatcaaaacttacttcaatgacaatgatcttaagtcgatgaatgtaaagggtgcctcccagggaatgtttatgacatacgcattagcccacgagttattgacgatcatcaaggaggtgataacctcttgtcaatccattgactccgtccccgaatacaacacagaagatatttggtttcagtttgcacttttaattctggaaaagaagaccggccacgtattcaacaagacaagcactctcacgtatatgccatgggaacgtaaactgcagtggacgaatgaacaaatagagtccgcaaagaggggcgaaaacattccggtaaacaagttcatcattaacagcattaccctttaa

SEQ ID NO: 4 - DNA, 2112 bp, Pasteurella multocida
  "Reencoded nucleic acid sequence of hyaluronan synthase (HASA) originating from Pasteurella multocida"
  Reencoded nucleic acid sequence of hyaluronan synthase (HASA) originating from Pasteurella multocida
atgaacaccctttcccaggcaattaaggcttataatagtaatgattatcaactagccctcaagctgttcgaaaagtcggcagaaatctacggcagaaagatagttgagttccaaattacgaagtgcaaggagaaactttctgcgcacccatccgttaacagtgcgcatctctcggttaacaaagaagagaaggtgaatgtttgcgacagtccattagacatagccactcaattattgttatcgaatgtgaaaaaactcgtccttagtgatagcgagaaaaatacactaaagaataaatggaagttgttgactgaaaagaagtctgagaacgcagaggtccgggccgtagctttagttcccaaggactttccgaaagatttagtgcttgcgccgttaccagaccatgtgaacgattttacgtggtataagaagcggaagaaacgcctaggaatcaaaccagaacaccaacacgttggcctctccattattgtgacaacgttcaaccgtcctgccatcctcagcatcaccctggcttgcctcgtcaatcaaaagacccattatccttttgaggtgatcgtgaccgacgatggttctcaagaggatttatcgcctataatccgtcaatatgagaacaagctagacatccgttatgttcggcaaaaggacaacggttttcaggcatcggccgcacgtaatatgggcctacgtctagccaaatatgacttcattgggctccttgattgtgatatggctcccaaccctttgtgggtacactcatacgttgcggaactattagaggacgatgatttgaccataataggccccaggaagtacattgacacgcaacacatagatcccaaggatttccttaataacgcctctctgttagagtcgttgccagaggttaagaccaataattccgtcgcggctaagggcgaggggaccgtatctttagactggcgtttggaacaatttgagaagaccgagaacttgaggctatccgatagccctttccgattcttcgcagctgggaatgtggctttcgccaagaagtggcttaacaagtcaggattcttcgacgaggaattcaatcactggggaggtgaagatgtagagttcggttatcgtctgtttcggtacggttcgttcttcaaaactatagacggcatcatggcctatcatcaggaaccgccaggtaaagaaaacgaaactgacagagaagcgggcaagaacattaccctcgatataatgagggagaaggtgccttacatctaccgtaaactcctgcctatagaagacagtcatatcaaccgagtaccattggtatcaatttacatcccggcctacaactgtgctaactatattcaaagatgtgttgattcagctttgaatcaaacggtagttgatctcgaagtgtgcatttgcaacgacggtagtactgacaacacgctggaagttattaacaagctgtatggtaataatccgcgtgtgcgtataatgtctaaacccaatggcggcattgcgagtgcatccaacgcagcggtcagcttcgcaaagggttattacataggacagttggacagcgacgattacttagaacccgacgcagtggagttatgtctcaaggaatttcttaaggataagacccttgcgtgcgtttacaccactaatcgtaacgtcaacccagatggctctttaatagccaatggctataactggccagagttcagtcgtgagaagttgactacggccatgattgctcatcacttccggatgtttaccattcgtgcttggcatctgacggatgggttcaatgagaagattgagaacgctgttgactacgacatgtttctcaagctcagtgaagttggtaaatttaagcatctgaacaaaatatgttataatcgggtgttacacggcgataacacctcaatcaagaagcttggcatacaaaagaagaatcatttcgtagttgtcaatcagtctctaaaccgccaaggtataacttattataactacgatgaatttgatgatctcgatgagagtcggaaatacattttcaacaagactgcagagtatcaagaagagatagatattcttaaagatatttaa

SEQ ID NO: 5 - DNA, 2322 bp, Pasteurella multocida
  "Reencoded nucleic acid sequence of hyaluronan synthase (HASA) originating from Pasteurella multocida"
  Reencoded nucleic acid sequence of hyaluronan synthase (HASA) originating from Pasteurella multocida
atgaacaccctttcccaggcaattaaggcttataatagtaatgattatcaactagccctcaagctgttcgaaaagtcggcagaaatctacggcagaaagatagttgagttccaaattacgaagtgcaaggagaaactttctgcgcacccatccgttaacagtgcgcatctctcggttaacaaagaagagaaggtgaatgtttgcgacagtccattagacatagccactcaattattgttatcgaatgtgaaaaaactcgtccttagtgatagcgagaaaaatacactaaagaataaatggaagttgttgactgaaaagaagtctgagaacgcagaggtccgggccgtagctttagttcccaaggactttccgaaagatttagtgcttgcgccgttaccagaccatgtgaacgattttacgtggtataagaagcggaagaaacgcctaggaatcaaaccagaacaccaacacgttggcctctccattattgtgacaacgttcaaccgtcctgccatcctcagcatcaccctggcttgcctcgtcaatcaaaagacccattatccttttgaggtgatcgtgaccgacgatggttctcaagaggatttatcgcctataatccgtcaatatgagaacaagctagacatccgttatgttcggcaaaaggacaacggttttcaggcatcggccgcacgtaatatgggcctacgtctagccaaatatgacttcattgggctccttgattgtgatatggctcccaaccctttgtgggtacactcatacgttgcggaactattagaggacgatgatttgaccataataggccccaggaagtacattgacacgcaacacatagatcccaaggatttccttaataacgcctctctgttagagtcgttgccagaggttaagaccaataattccgtcgcggctaagggcgaggggaccgtatctttagactggcgtttggaacaatttgagaagaccgagaacttgaggctatccgatagccctttccgattcttcgcagctgggaatgtggctttcgccaagaagtggcttaacaagtcaggattcttcgacgaggaattcaatcactggggaggtgaagatgtagagttcggttatcgtctgtttcggtacggttcgttcttcaaaactatagacggcatcatggcctatcatcaggaaccgccaggtaaagaaaacgaaactgacagagaagcgggcaagaacattaccctcgatataatgagggagaaggtgccttacatctaccgtaaactcctgcctatagaagacagtcatatcaaccgagtaccattggtatcaatttacatcccggcctacaactgtgctaactatattcaaagatgtgttgattcagctttgaatcaaacggtagttgatctcgaagtgtgcatttgcaacgacggtagtactgacaacacgctggaagttattaacaagctgtatggtaataatccgcgtgtgcgtataatgtctaaacccaatggcggcattgcgagtgcatccaacgcagcggtcagcttcgcaaagggttattacataggacagttggacagcgacgattacttagaacccgacgcagtggagttatgtctcaaggaatttcttaaggataagacccttgcgtgcgtttacaccactaatcgtaacgtcaacccagatggctctttaatagccaatggctataactggccagagttcagtcgtgagaagttgactacggccatgattgctcatcacttccggatgtttaccattcgtgcttggcatctgacggatgggttcaatgagaagattgagaacgctgttgactacgacatgtttctcaagctcagtgaagttggtaaatttaagcatctgaacaaaatatgttataatcgggtgttacacggcgataacacctcaatcaagaagcttggcatacaaaagaagaatcatttcgtagttgtcaatcagtctctaaaccgccaaggtataacttattataactacgatgaatttgatgatctcgatgagagtcggaaatacattttcaacaagactgcagagtatcaagaagagatagatattcttaaagatattggatccgccatttctcaaatcactgacggtcaaatccaagctactaccactgctaccaccgaagctaccaccactgctgccccatcttccaccgttgaaactgtttctccatccagcaccgaaactatctctcaacaaactgaaaatggtgctgctaaggccgctgtcggtatgggtgccggtgctctagctgctgctgctatgttgttataa

SEQ ID NO: 6 - DNA, 1656 bp, Xenopus laevis
  "Reencoded nucleic acid sequence of hyaluronan synthase (HASA) originating from Xenopus laevis"
  Reencoded nucleic acid sequence of hyaluronan synthase (HASA) originating from Xenopus laevis
atgcactgtgaacgatttatttgtatattacgaataattggtacgactttgttcggagtaagtctgctactagggatatccgccgcttatatcgtgggataccaattcattcagacggataattactacttttccttcggtctctacggtgctattttagctttacatttaatcattcagtctctcttcgcattcctggagcatcgtaagatgaagcggtcacttgaaacccctataaaattaaacaagagcgtagcattgtgtatcgctgcataccaggaagacgaagattatcttagaaaatgtttgctttctgtgaaacggctcacataccccggtatgaaggtaatcatggtgatagatggtaactctgatgacgatctatacatgatgaacatattcagagagatcatgggaaatgatagctgcgccacctatgtatggaagaataattttcacatgaagggaccaaacgagaccgacgagactcaccgcgagtccatgcagcatgtaacacagatggtgctttctaacagaaatgtctgtatcatgcaaaagtggaacgggaaacgcgaggtgatgtatactgcattcaaagcgctgggtcggtcggttgattacgtccaagtgtgcgactcagatacagtccttgatccagcaagctcggtggagatggtcaaggtgttggaggaagacattatggtcggaggtgtaggcggagacgtgcagatactcaataagtacgactcctggatcagtttcttgagttcggttcgttattggatggctttcaatatagaacgagcatgccaatcatactttggctgtgtgcagtgtatatcggggcctctgggcatgtacagaaactcactcttacatgagttcattgaagactggtacaatcaagaattcctcggttcccaatgctctttcggtgatgatcggcatttgactaatcgagtactatcattgggctatgctactaaatacactgcgcgcagtaagtgtctgacagaaacccccacagaatatcttagatggttgaaccaacaaaccaggtggagtaagtcctatttccgcgagtggttgtacaactctttgtggttccacaaacaccatttatggatgacttatgaagccgtaattacgggtttcttccccttcttcttaatagcgacggtgattcagctcttctatcgtggtcgaatttggaatatcttactctttctactcacagttcaattagttggtctaataaagtcgtcgtttgcaagtgcgttgcgtggaaacatcgttatggtctttatgagtttctacagtgttttatacatgagtagcttgctgccagcaaagatgtttgcaatcgccacgataaacaaggctggatggggtactagtggtagaaagaccatagttgttaattttattggtttaatccctattacggtatggttcacaattttactagggggagtatgctacactatatggcgggaaaccaagaagccgtttagcgagtctgagaagatcgttcttgcggtcggtgctatattgtatgcttgttattgggtcatgttgcttacaatgtatgtcagtcttgtcatgaagtgcgggcgccgtaggaaggaaccacagcacgaccttgttttagcataa

SEQ ID NO: 7 - DNA, 1254 bp, Streptococcus zooepidemicus
  "Reencoded nucleic acid sequence of hyaluronan synthase (HASA) originating from Streptococcus zooepidemicus"
  Reencoded nucleic acid sequence of hyaluronan synthase (HASA) originating from Streptococcus zooepidemicus
atgaggacgttaaagaatcttatcactgttgtagcgttcagtatattctgggttttgctgatctatgtaaatgtctatcttttcggtgcgaaggggtctctatcaatatatggattcttgctaattgcgtatttgcttgtgaagatgagtctttcattcttctataaaccattcaaaggtcgagctggtcagtataaagtcgcagcgattatcccttcatacaacgaggatgcagaatcgctgttggaaaccttaaaatctgttcaacaacaaacctatccccttgctgaaatttatgtagttgatgatggttccgcagatgaaaccggtatcaagcggatcgaggattatgtcagggatacaggcgacttaagttcaaatgtgattgtgcatcgatcagaaaagaatcaaggcaagagacacgcccaagcatgggcatttgaaagatctgatgcagatgtatttctaacagtcgatagtgatacttacatttatccggacgcccttgaagagttattgaaaaccttcaatgatccgacagtatttgccgcaactggccacttgaacgttcgtaacaggcagactaatctattgaccagactcactgatataagatacgacaatgcttttggcgtcgaacgtgctgctcaaagtgtaactggtaatatactggtgtgttccgggccactgtccgtctatcgcagagaagtagtagtcccgaacattgacaggtatattaatcagacttttctgggtatccccgtgtcaattggggacgaccggtgtttaacgaactacgctactgatttgggcaagactgtatatcagtcgacggctaaatgtattacagacgtcccagataagatgtcgacttaccttaaacagcagaatagatggaataagtcattctttagagaatctatcatcagcgtgaagaagatcatgaataatccattcgtggcgctttggaccattttggaggtttccatgtttatgatgcttgtctactctgtcgttgatttctttgtaggtaacgttcgagaatttgattggctcagagttcttgctttcttagttatcatcttcatcgttgcgctatgcaggaatattcattacatgctaaaacatccgcttagcttcttactcagccctttctacggcgttttgcatctcttcgttttgcagccattgaagctctactccttatttaccattcgaaacgctgattggggtacgcgcaagaaactattataa

SEQ ID NO: 8 - protein, 568 aa, Paramecium bursaria Chlorella virus 1
  Amino acid sequence of hyaluronan synthase (HASA) originating from Chlorella virus PBCV-1
  Amino acid sequence of hyaluronan synthase (HASA) originating from Chlorella virus PBCV-1
MGKNIIIMVSWYTIITSNLIAVGGASLILAPAITGYVLHWNIALSTIWGVSAYGIFVFGFFLAQVLFSELNRKRLRKWISLRPKGWNDVRLAVIIAGYREDPYMFQKCLESVRDSDYGNVARLICVIDGDEDDDMRMAAVYKAIYNDNIKKPEFVLCESDDKEGERIDSDFSRDICVLQPHRGKRECLYTGFQLAKMDPSVNAVVLIDSDTVLEKDAILEVVYPLACDPEIQAVAGECKIWNTDTLLSLLVAWRYYSAFCVERSAQSFFRTVQCVGGPLGAYKIDIIKEIKDPWISQRFLGQKCTYGDDRRLTNEILMRGKKVVFTPFAVGWSDSPTNVFRYIVQQTRWSKSWCREIWYTLFAAWKHGLSGIWLAFECLYQITYFFLVIYLFSRLAVEADPRAQTATVIVSTTVALIKCGYFSFRAKDIRAFYFVLYTFVYFFCMIPARITAMMTLWDIGWGTRGGNEKPSVGTRVALWAKQYLIAYMWWAAVVGAGVYSIVHNWMFDWNSLSYRFALVGICSYIVFIVIVLVVYFTGKITTWNFTKLQKELIEDRVLYDATTNAQSV

SEQ ID NO: 9 - protein, 972 aa, Pasteurella multocida
  Amino acid sequence of hyaluronan synthase (HASA) originating from Pasteurella multocida
  Amino acid sequence of hyaluronan synthase (HASA) originating from Pasteurella multocida
MNTLSQAIKAYNSNDYQLALKLFEKSAEIYGRKIVEFQITKCKEKLSAHPSVNSAHLSVNKEEKVNVCDSPLDIATQLLLSNVKKLVLSDSEKNTLKNKWKLLTEKKSENAEVRAVALVPKDFPKDLVLAPLPDHVNDFTWYKKRKKRLGIKPEHQHVGLSIIVTTFNRPAILSITLACLVNQKTHYPFEVIVTDDGSQEDLSPIIRQYENKLDIRYVRQKDNGFQASAARNMGLRLAKYDFIGLLDCDMAPNPLWVHSYVAELLEDDDLTIIGPRKYIDTQHIDPKDFLNNASLLESLPEVKTNNSVAAKGEGTVSLDWRLEQFEKTENLRLSDSPFRFFAAGNVAFAKKWLNKSGFFDEEFNHWGGEDVEFGYRLFRYGSFFKTIDGIMAYHQEPPGKENETDREAGKNITLDIMREKVPYIYRKLLPIEDSHINRVPLVSIYIPAYNCANYIQRCVDSALNQTVVDLEVCICNDGSTDNTLEVINKLYGNNPRVRIMSKPNGGIASASNAAVSFAKGYYIGQLDSDDYLEPDAVELCLKEFLKDKTLACVYTTNRNVNPDGSLIANGYNWPEFSREKLTTAMIAHHFRMFTIRAWHLTDGFNEKIENAVDYDMFLKLSEVGKFKHLNKICYNRVLHGDNTSIKKLGIQKKNHFVVVNQSLNRQGITYYNYDEFDDLDESRKYIFNKTAEYQEEIDILKDIKIIQNKDAKIAVSIFYPNTLNGLVKKLNNIIEYNKNIFVIVLHVDKNHLTPDIKKEILAFYHKHQVNILLNNDISYYTSNRLIKTEAHLSNINKLSQLNLNCEYIIFDNHDSLFVKNDSYAYMKKYDVGMNFSALTHDWIEKINAHPPFKKLIKTYFNDNDLKSMNVKGASQGMFMTYALAHELLTIIKEVITSCQSIDSVPEYNTEDIWFQFALLILEKKTGHVFNKTSTLTYMPWERKLQWTNEQIESAKRGENIPVNKFIINSITL

SEQ ID NO: 10 - protein, 551 aa, Xenopus laevis
  Amino acid sequence of hyaluronan synthase (HASA) originating from Xenopus laevis
  Amino acid sequence of hyaluronan synthase (HASA) originating from Xenopus laevis
MHCERFICILRIIGTTLFGVSLLLGISAAYIVGYQFIQTDNYYFSFGLYGAILALHLIIQSLFAFLEHRKMKRSLETPIKLNKSVALCIAAYQEDEDYLRKCLLSVKRLTYPGMKVIMVIDGNSDDDLYMMNIFREIMGNDSCATYVWKNNFHMKGPNETDETHRESMQHVTQMVLSNRNVCIMQKWNGKREVMYTAFKALGRSVDYVQVCDSDTVLDPASSVEMVKVLEEDIMVGGVGGDVQILNKYDSWISFLSSVRYWMAFNIERACQSYFGCVQCISGPLGMYRNSLLHEFIEDWYNQEFLGSQCSFGDDRHLTNRVLSLGYATKYTARSKCLTETPTEYLRWLNQQTRWSKSYFREWLYNSLWFHKHHLWMTYEAVITGFFPFFLIATVIQLFYRGRIWNILLFLLTVQLVGLIKSSFASALRGNIVMVFMSFYSVLYMSSLLPAKMFAIATINKAGWGTSGRKTIVVNFIGLIPITVWFTILLGGVCYTIWRETKKPFSESEKIVLAVGAILYACYWVMLLTMYVSLVMKCGRRRKEPQHDLVLA

SEQ ID NO: 11 - protein, 417 aa, Streptococcus zooepidemicus
  Amino acid sequence of hyaluronan synthase (HASA) originating from Streptococcus zooepidemicus
  Amino acid sequence of hyaluronan synthase (HASA) originating from Streptococcus zooepidemicus
MRTLKNLITVVAFSIFWVLLIYVNVYLFGAKGSLSIYGFLLIAYLLVKMSLSFFYKPFKGRAGQYKVAAIIPSYNEDAESLLETLKSVQQQTYPLAEIYVVDDGSADETGIKRIEDYVRDTGDLSSNVIVHRSEKNQGKRHAQAWAFERSDADVFLTVDSDTYIYPDALEELLKTFNDPTVFAATGHLNVRNRQTNLLTRLTDIRYDNAFGVERAAQSVTGNILVCSGPLSVYRREVVVPNIDRYINQTFLGIPVSIGDDRCLTNYATDLGKTVYQSTAKCITDVPDKMSTYLKQQNRWNKSFFRESIISVKKIMNNPFVALWTILEVSMFMMLVYSVVDFFVGNVREFDWLRVLAFLVIIFIVALCRNIHYMLKHPLSFLLSPFYGVLHLFVLQPLKLYSLFTIRNADWGTRKKLL

SEQ ID NO: 12 - DNA, 1446 bp, Arabidopsis thaliana
  "Nucleic acid sequence of UDP-Glucose dehydrogenase (HASB) originating from Arabidopsis thaliana"
  Nucleic acid sequence of UDP-Glucose dehydrogenase (HASB) originating from Arabidopsis thaliana
atggtcaaaatatgctgtatcggggctggatatgtcggtgggcctacaatggccgttatggccctaaagtgtccagagattgaagtcgtggtagttgatatatcggagccacgaattaacgcatggaactcagaccgtctaccaatttatgagccagggttagaggatgtcgtcaaacagtgtagagggaagaatttgttcttctctacagatgtagagaagcatgtatttgagtcagatatagtgtttgtttcggtaaacactcctacgaaaacgcagggtctgggtgcaggtaaagcagcagatttgacatattgggagtccgctgctcgcatgatagctgatgtgagcaaatcgtcgaaaatcgtcgttgaaaagagtacagtaccagttcgtacagccgaggctatagaaaagattttaacgcacaattcgaagggtatcgaattccagatcttatcaaatccagaattcttggccgaagggacggcgattaaagacttatataaccctgatagagttctaatcggtggcagggacaccgctgcgggacaaaaggccattaaggcgttgcgtgacgtgtatgcccactgggttcctgttgagcaaataatctgtactaatttatggagtgccgagctatcaaagttggctgcgaacgcatttctagctcaaaggataagttcagtaaacgcaatgtcagcgctttgtgaggcaactggtgctgacgtaacccaagtcgctcacgccgttggaaccgacactagaattggaccgaagtttcttaacgcatccgtaggcttcggcggatcttgctttcagaaagacatcctgaatcttatttacatctgcgaatgcaatggtcttccagaagcagccaattattggaaacaggtagtcaaggtaaatgactaccaaaagattaggtttgctaatcgagtcgtatcttctatgttcaacaccgtctccggtaagaaaattgctattttgggatttgcgttcaagaaggacaccggcgacacgcgtgaaactcctgccatagatgtgtgtaatcgcctcgtggctgataaagcaaagctgtcgatctatgatccgcaagtattagaagagcagatccgccgtgatctgtccatggcccgattcgattgggaccatccagtcccactccagcagatcaaagctgaaggtatctccgaacaggttaacgttgtgtccgacgcctacgaggctacgaaggatgctcatggtttatgtgttttaaccgaatgggacgaattcaagtcacttgattttaagaagatctttgataatatgcagaaacccgctttcgttttcgacggaagaaacgtggtcgacgctgtgaaattgagagaaattggattcatagtatattccataggtaaacctctggatagttggctcaaggatatgccggctgttgcataa

SEQ ID NO: 13 - DNA, 1166 bp, Paramecium bursaria Chlorella virus 1
  "Reencoded nucleic acid sequence of UDP-Glucose dehydrogenase (HASB) originating from Chlorella virus PBCV-1"
  Reencoded nucleic acid sequence of UDP-Glucose dehydrogenase (HASB) originating from Chlorella virus PBCV-1
atgagtagaattgctgtcgttggatgcggttacgtgggtacggcctgcgccgtacttttggcgcagaagaacgaagttatcgttttggatatctcggaggaccgggtacaactgattaagaataagaagtcacctatagaagataaggaaatcgaagaattcctggagacgaaagatttgaatctaacagcgacgacggataaggtgctcgcctatgagaatgctgaattcgttataatagctacaccgaccgattacgatgtcgtcactagatatttcaacactaagtctgttgaaaatgtgataggcgatgtcattaagaacactcagacacaccctactatagtgatcaagagtactattccaatcggtttcgtggataaagttagagaacagttcgattatcaaaatattatcttctcgccggaattcttgagagaaggacgagcattatatgataatctttacccctcccgtatcatcgtcggtgatgactccccaattgccttaaaattcgcgaatctcttggtcgagggtagcaaaactccactagctcccgtattaactatgggtacgcgagaggccgaagctgtaaaactattttcaaatacatatttggctatgagagtagcatacttcaatgagctagacacatttgcaatgtcccatggtatgaacgcaaaagagattatcgacggagtcacactagaaccaaggatagggcagggttattcgaatccttcatttgggtatggagcctattgtttcccaaaagatacaaagcaattgttggctaattttgaaggggttccacaagatattattggcgcaatcgtagagtctaacgaaactagaaaggaggttattgtttctgaggtcgagaacagatttccgaccacagttggcgtatataagttggctgctaaagctggttcggataatttcaggtctagtgcgatagtcgatatcatggaaaggttggctaataagggctaccacatcaaaatatttgaacctaccgttgaacaatttgagaattttgaggtagataataatctcacaacttttgcaaccgagtctgatgtaataattgcgaacagagttccagtcgaacatcgcattctgtttgggaagaagttaataacacgggatgtctatggggataa

SEQ ID NO: 14 - DNA, 1170 bp, Paramecium bursaria Chlorella virus 1
  "Reencoded nucleic acid sequence of UDP-Glucose dehydrogenase (HASB) originating from Chlorella virus PBCV-1"
  Reencoded nucleic acid sequence of UDP-Glucose dehydrogenase (HASB) originating from Chlorella virus PBCV-1
atgtcacgaatcgcagtagttggctgtgggtacgtgggaaccgcatgcgctgtactgctggcgcaaaagaatgaggtaatcgttcttgatattagtgaggatagggtccaactaatcaagaacaagaaatccccgatcgaagataaggagattgaagaattcttggaaacaaaagacctaaacttaactgcaacaactgacaaagttttagcctacgaaaacgctgagtttgtgattatagcgacacccacagattatgacgtagttaccagatactttaacacgaagtccgtagagaacgtcattggagatgttataaagaatactcagactcatcctacgatagtaataaagtcaaccattcccataggtttcgtagataaggttagggagcaattcgattaccagaacattatattttcgccagaatttctgagagagggtcgcgccctgtatgataatctatatccatcacggattatagtgggcgatgactctccgattgcacttaagtttgctaatcttttagttgagggctccaaaactccgctcgccccagtacttacgatgggtacacgtgaggctgaagctgtcaagctgttttcaaacacataccttgctatgcgagtcgcatactttaacgaactagatacctttgctatgtcgcacggtatgaatgctaaagaaatcatagatggcgtaacgttggagcctcggataggtcaaggatattccaatccatcttttggctacggtgcgtattgtttcccaaaggacacgaagcaattattagctaactttgagggtgttccgcaagatataattggggcgatagtagaaagcaatgaaacacggaaggaggtaatcgtgagtgaagtggaaaaccgattccccactacggtcggcgtttacaaattagccgccaaggctggttccgacaatttccgatccagcgcaatagtagatattatggaaagattagctaataagggataccacattaaaatctttgaacctactgtcgaacagttcgagaacttcgaggttgataataacttgacgactttcgcaacggagagcgatgtaattattgcaaaccgcgtacctgtggaacatcgaattttgttcggaaagaagctgattacacgcgatgtatatggcgataactaa

SEQ ID NO: 15 - DNA, 1199 bp, streptococcus zooepidemicus
  "Reencoded nucleic acid sequence of UDP-Glucose dehydrogenase (HASB) originating from Streptococcus zooepidemicus"
  Reencoded nucleic acid sequence of UDP-Glucose dehydrogenase (HASB) originating from Streptococcus zooepidemicus
atgaagatatcggtagcgggttcggggtacgtggggttatccttgtcaatcttgcttgcccaacataacgatgtgactgttgtagatataatcgacgaaaaggtacggctaattaaccagggcatatctccgattaaggatgcggacattgaggaatatctgaagaatgcaccgttgaatcttacggctacactagacggagcttcggcttatagtaatgctgatctgattataatcgcaacgccaactaattacgattcagaacgcaattatttcgacaccagacacgttgaagaagtaattgagcaagtattggatttaaatgcctccgctactataatcatcaagagtaccatacccttgggttttattaaacacgtaagagagaaataccaaacagacagaatcatcttttctccagagttcttaagagagtcaaaggcattgtacgataacttatacccctctcgtataatagtcagttatgagaaggatgactctccaagagttatacaagcagctaaggcgttcgcgggtttattaaaagagggggcaaagagcaaggataccccagttctgtttatgggctctcaagaagctgaagctgtcaagctgtttgctaatacttttctcgccatgagggtcagttacttcaacgagcttgacacttatagcgaatcaaaaggactagacgcccaaagagttatagaaggcgtctgccatgatcaaaggataggtaatcattacaataatccatccttcggatatggcggttattgtttacccaaagactcaaagcaacttttggctaattatagaggcatacctcagtctctaatgtctgccatcgttgaatcgaacaagatccgtaagtcgtatttagctgaacaaatattagatagggcttcttcacaaaagcaggctggtgtacctttaaccataggattttaccgtttgattatgaagtccaactccgataactttagagaatcagccattaaagatattattgacatcattaatgactacggtgtcaatattgtcatttatgaacctatgttgggagaagacattggttatagagtcgttaaagatttggaacagtttaagaacgaaagtacaattattgttagtaacaggtttgaagatgatttaggtgatgttattgataaagtttatacacgtgacgtctttggtag

SEQ ID NO: 16 - protein, 481 aa, Arabidopsis thaliana
  Amino acid sequence of UDP-Glucose dehydrogenase (HASB) originating from Arabidopsis thaliana
  Amino acid sequence of UDP-Glucose dehydrogenase (HASB) originating from Arabidopsis thaliana
MVKICCIGAGYVGGPTMAVMALKCPEIEVVVVDISEPRINAWNSDRLPIYEPGLEDVVKQCRGKNLFFSTDVEKHVFESDIVFVSVNTPTKTQGLGAGKAADLTYWESAARMIADVSKSSKIVVEKSTVPVRTAEAIEKILTHNSKGIEFQILSNPEFLAEGTAIKDLYNPDRVLIGGRDTAAGQKAIKALRDVYAHWVPVEQIICTNLWSAELSKLAANAFLAQRISSVNAMSALCEATGADVTQVAHAVGTDTRIGPKFLNASVGFGGSCFQKDILNLIYICECNGLPEAANYWKQVVKVNDYQKIRFANRVVSSMFNTVSGKKIAILGFAFKKDTGDTRETPAIDVCNRLVADKAKLSIYDPQVLEEQIRRDLSMARFDWDHPVPLQQIKAEGISEQVNVVSDAYEATKDAHGLCVLTEWDEFKSLDFKKIFDNMQKPAFVFDGRNVVDAVKLREIGFIVYSIGKPLDSWLKDMPAVA

SEQ ID NO: 17 - protein, 389 aa, Paramecium bursaria Chlorella virus 1
  Amino acid sequence of UDP-Glucose dehydrogenase (HASB) originating from Chlorella virus PBCV1
  Amino acid sequence of UDP-Glucose dehydrogenase (HASB) originating from Chlorella virus PBCV1
MSRIAVVGCGYVGTACAVLLAQKNEVIVLDISEDRVQLIKNKKSPIEDKEIEEFLETKDLNLTATTDKVLAYENAEFVIIATPTDYDVVTRYFNTKSVENVIGDVIKNTQTHPTIVIKSTIPIGFVDKVREQFDYQNIIFSPEFLREGRALYDNLYPSRIIVGDDSPIALKFANLLVEGSKTPLAPVLTMGTREAEAVKLFSNTYLAMRVAYFNELDTFAMSHGMNAKEIIDGVTLEPRIGQGYSNPSFGYGAYCFPKDTKQLLANFEGVPQDIIGAIVESNETRKEVIVSEVENRFPTTVGVYKLAAKAGSDNFRSSAIVDIMERLANKGYHIKIFEPTVEQFENFEVDNNLTTFATESDVIIANRVPVEHRILFGKKLITRDVYGDN

SEQ ID NO: 18 - protein, 401 aa, Streptococcus zooepidemicus
  Amino acid sequence of UDP-Glucose dehydrogenase (HASB) originating from Streptococcus zooepidemicus
  Amino acid sequence of UDP-Glucose dehydrogenase (HASB) originating from Streptococcus zooepidemicus
MKISVAGSGYVGLSLSILLAQHNDVTVVDIIDEKVRLINQGISPIKDADIEEYLKNAPLNLTATLDGASAYSNADLIIIATPTNYDSERNYFDTRHVEEVIEQVLDLNASATIIIKSTIPLGFIKHVREKYQTDRIIFSPEFLRESKALYDNLYPSRIIVSYEKDDSPRVIQAAKAFAGLLKEGAKSKDTPVLFMGSQEAEAVKLFANTFLAMRVSYFNELDTYSESKGLDAQRVIEGVCHDQRIGNHYNNPSFGYGGYCLPKDSKQLLANYRGIPQSLMSAIVESNKIRKSYLAEQILDRASSQKQAGVPLTIGFYRLIMKSNSDNFRESAIKDIIDIINDYGVNIVIYEPMLGEDIGYRVVKDLEQFKNESTIIVSNRFEDDLGDVIDKVYTRDVFGRD

SEQ ID NO: 19 - DNA, 1326 bp, Bothrops atrox
  "Reencoded nucleic acid sequence of hyaluronidase (HYAL) originating from Bothrops atrox with a N-terminal secretion signal"
  Reencoded nucleic acid sequence of hyaluronidase (HYAL) originating from Bothrops atrox with a N-terminal secretion signal
atgcaatttagcacagtcgcatcagtagccttcgttgccttggccaacttcgtggcagcaccgatgtatccgaacgaaccgttcttagtcttttggaacgcgcctacaactcagtgtagacttcgatataaggttgaccttgatctgaagacattccatatcgtgacaaatgctaatgactcgctgtcaggatcggctgtcacgattttctatcccacgcacttaggggtttacccacatattgatgacagggggcacttcttcaatggcatcataccccaaaatgaatccctggtaaagcatttaaacaaatctaaatcagatattaatcgaatgattcccttaagaacattccacgggctgggagtcatagactgggaaaactggcggccacagtgggataggaattggggaagtaagaacgtttataggaatagatcaatccaattcgcgcgtgatctccacccagagcttagtgaggacaagattaaacgcttggcaaaacaggaattcgagaaagctgcaaagagttttatgagggatacactattattagccgaggagatgcgaccagacggctactggggatactatctgtaccccgattgtcacaattacaattataagactaagccagatcagtacacaggagagtgccctgacatcgagatgtcacgtaacaatcaactcttgtggctttggcgggatagcactgcccttttccccaatatctacttagagactatactaagaagctctgacaatgccctgaagtttgtgcaccataggctcaaggaggcaatgaggatagcctcaatggctcgaaatgactacgcgttgcctttctttgtttatgctcgaccattctatgcctataccttcgaaccattgactcaggaagaccttgtgactacggtcggagagaccgcggacatgggcgccgctgggatcgtattttgggggagtatgcagtacgcaagcacggttgaatcttgcggcaaagtcaaggactacatgaatggcccactggggcgttacattgtgaatgttacaactgccgccaaaatttgctcacgattcttgtgcaaacgtcatggtaggtgtgtaagaaagcactcagactccaatgcattccttcacctatttcccgattcgtttcgcataatggtgcacgggaatgcaaccgagaagaaagttatagtaaaggggaagctggaattaaagaatcttatattcttacgtaataactttatgtgccagtgttatcaaggctggaaaggtctatattgcgagaagcattcgataaaggaaattcggaaaatctaa

SEQ ID NO: 20 - DNA, 1537 bp, Bothrops atrox
  "Reencoded nucleic acid sequence of hyaluronidase (HYAL) originating from Bothrops atrox with a N-terminal secretion signal and a C-terminal anchoring signal"
  Reencoded nucleic acid sequence of hyaluronidase (HYAL) originating from Bothrops atrox with a N-terminal secretion signal and a C-terminal anchoring signal
atgcaatttagcacagtcgcatcagtagccttcgttgccttggccaacttcgtggcagcaccgatgtatccgaacgaaccgttcttagtcttttggaacgcgcctacaactcagtgtagacttcgatataaggttgaccttgatctgaagacattccatatcgtgacaaatgctaatgactcgctgtcaggatcggctgtcacgattttctatcccacgcacttaggggtttacccacatattgatgacagggggcacttcttcaatggcatcataccccaaaatgaatccctggtaaagcatttaaacaaatctaaatcagatattaatcgaatgattcccttaagaacattccacgggctgggagtcatagactgggaaaactggcggccacagtgggataggaattggggaagtaagaacgtttataggaatagatcaatccaattcgcgcgtgatctccacccagagcttagtgaggacaagattaaacgcttggcaaaacaggaattcgagaaagctgcaaagagttttatgagggatacactattattagccgaggagatgcgaccagacggctactggggatactatctgtaccccgattgtcacaattacaattataagactaagccagatcagtacacaggagagtgccctgacatcgagatgtcacgtaacaatcaactcttgtggctttggcgggatagcactgcccttttccccaatatctacttagagactatactaagaagctctgacaatgccctgaagtttgtgcaccataggctcaaggaggcaatgaggatagcctcaatggctcgaaatgactacgcgttgcctttctttgtttatgctcgaccattctatgcctataccttcgaaccattgactcaggaagaccttgtgactacggtcggagagaccgcggacatgggcgccgctgggatcgtattttgggggagtatgcagtacgcaagcacggttgaatcttgcggcaaagtcaaggactacatgaatggcccactggggcgttacattgtgaatgttacaactgccgccaaaatttgctcacgattcttgtgcaaacgtcatggtaggtgtgtaagaaagcactcagactccaatgcattccttcacctatttcccgattcgtttcgcataatggtgcacgggaatgcaaccgagaagaaagttatagtaaaggggaagctggaattaaagaatcttatattcttacgtaataactttatgtgccagtgttatcaaggctggaaaggtctatattgcgagaagcattcgataaaggaaattcggaaaatcggatccgccatttctcaaatcactgacggtcaaatccaagctactaccactgctaccaccgaagctaccaccactgctgccccatcttccaccgttgaaactgtttctccatccagcaccgaaactatctctcaacaaactgaaaatggtgctgctaaggccgctgtcggtatgggtgccggtgctctagctgctgctgctatgttgttataaa

SEQ ID NO: 21 - DNA, 1197 bp, Cupiennius salei
  "Reencoded nucleic acid sequence of hyaluronidase (HYAL) originating from Cupiennius salei with a N-terminal secretion signal"
  Reencoded nucleic acid sequence of hyaluronidase (HYAL) originating from Cupiennius salei with a N-terminal secretion signal
atgcaattcagcactgttgcatcagttgcatttgtcgccctggcgaattttgtagccgcgttcaagatttactggaacgtcccaacttttcagtgcacgcataactacaaaatcgattatgtcaaattgttgtccacttacgggatacaggtcaatgatggcggtaagtttcaaggaaaccaagtgactatcttttatgaaacccagttgggtttgtatccacgaatcctaaaatctggtaaaatggaaaacggcggaatccctcaacgcggtaactttgagaaacacctagaaaaggcaagcacggacctccagaaagtgatcccttggaaagagtttagcggattaggtgtgatagattgggaggcttggagacccacatgggaatttaactgggaaccgttgaggatatatcaaaccgaatcaattaagagagctaaagaactacaccctaccgcaaacgattccgcagtaaaagaaattgcagagcggcaatgggaagattcagccaagttatacatgttagaaacactgcggctggcaaagaaacttcgacctcaagcgccttggtgttactacttatttcctgattgctataattacgtcggaaagaaaccaaaagatttccaatgtagtgcctcgatacgtaaaggtaacgataagctaagctggttgtggaaagattctacggcattgtgtccatcgatatacgtatatgaatcacaattagacaggtattcttttgaacaaaggacatggcgcgacaatgagaaacttcgggaagcgttgcgtgtagccacgagaacctctaaaatatacccatacgttaactatttcgataaggagcttataccggagcaagaagtatggagaatgcttgcgcaggcagctgctgtcggtggcagtggtgcggtaatttggggctcatctgctgcagttgcatctgaagagttatgtaaatctttaaaacagtatattattgaaacgcttgggccggcggcagagaaggtggcttggcgtagtgacttatgcagcaaagaaatttgtaataatcagggtcgctgcacattcccggacgatgattatgcaaacgcatggaaattatttacagatgatactgttaagttttatgctggtaatattacatgtaggtgctccgagaattattctggtcgtttctgcgaaaagaagaattaa

SEQ ID NO: 22 - DNA, 1407 bp, Cupiennius salei
  "Reencoded nucleic acid sequence of hyaluronidase (HYAL) originating from Cupiennius salei with a N-terminal secretion signal and a C-terminal anchoring signal"
  Reencoded nucleic acid sequence of hyaluronidase (HYAL) originating from Cupiennius salei with a N-terminal secretion signal and a C-terminal anchoring signal
atgcaattcagcactgttgcatcagttgcatttgtcgccctggcgaattttgtagccgcgttcaagatttactggaacgtcccaacttttcagtgcacgcataactacaaaatcgattatgtcaaattgttgtccacttacgggatacaggtcaatgatggcggtaagtttcaaggaaaccaagtgactatcttttatgaaacccagttgggtttgtatccacgaatcctaaaatctggtaaaatggaaaacggcggaatccctcaacgcggtaactttgagaaacacctagaaaaggcaagcacggacctccagaaagtgatcccttggaaagagtttagcggattaggtgtgatagattgggaggcttggagacccacatgggaatttaactgggaaccgttgaggatatatcaaaccgaatcaattaagagagctaaagaactacaccctaccgcaaacgattccgcagtaaaagaaattgcagagcggcaatgggaagattcagccaagttatacatgttagaaacactgcggctggcaaagaaacttcgacctcaagcgccttggtgttactacttatttcctgattgctataattacgtcggaaagaaaccaaaagatttccaatgtagtgcctcgatacgtaaaggtaacgataagctaagctggttgtggaaagattctacggcattgtgtccatcgatatacgtatatgaatcacaattagacaggtattcttttgaacaaaggacatggcgcgacaatgagaaacttcgggaagcgttgcgtgtagccacgagaacctctaaaatatacccatacgttaactatttcgataaggagcttataccggagcaagaagtatggagaatgcttgcgcaggcagctgctgtcggtggcagtggtgcggtaatttggggctcatctgctgcagttgcatctgaagagttatgtaaatctttaaaacagtatattattgaaacgcttgggccggcggcagagaaggtggcttggcgtagtgacttatgcagcaaagaaatttgtaataatcagggtcgctgcacattcccggacgatgattatgcaaacgcatggaaattatttacagatgatactgttaagttttatgctggtaatattacatgtaggtgctccgagaattattctggtcgtttctgcgaaaagaagaatggatccgccatttctcaaatcactgacggtcaaatccaagctactaccactgctaccaccgaagctaccaccactgctgccccatcttccaccgttgaaactgtttctccatccagcaccgaaactatctctcaacaaactgaaaatggtgctgctaaggccgctgtcggtatgggtgccggtgctctagctgctgctgctatgttgttataa

SEQ ID NO: 23 - DNA, 1530 bp, Hirudo nipponia
  "Reencoded nucleic acid sequence of hyaluronidase (HYAL) originating from Hirudo Nipponia with a N-terminal secretion signal"
  Reencoded nucleic acid sequence of hyaluronidase (HYAL) originating from Hirudo Nipponia with a N-terminal secretion signal
atgcaattctctactgtcgcttccgttgctttcgtcgctttggctaactttgttgccgctatgaaggagatagcagttaccatcgatgataagaatgttatagcgtctgtcagtgaaagcttccatggtgtggctttcgacgcaagcctattctcacctaaagggctatggtcgtttgttgacattacttcacccaagttattcaagcttctggagggactctcccctggttatttccgtgtcggcggcacatttgcgaactggttattcttcgacctcgatgaaaacaacaagtggaaggattactgggcttttaaggacaagactccagagaccgccacgattacccgacggtggctcttcaggaagcaaaacaacctcaagaaggaaacctttgatgatttggtaaagcttacaaaggggtccaagatgcggctgctatttgatctaaacgcagaggtccgtacaggatatgagataggcaagaagatgacatcaacttgggactcaagcgaggcagaaaagttgttcaaatattgcgttagcaagggatatggagataatatcgattgggagttaggcaacgaacctgatcacacgtcagcacacaatttgacagagaagcaagtaggtgaagattttaaggccctacacaaggtgttggaaaagtatccaacacttaataaaggtagcttggttggtccagacgttgggtggatgggagtgtcgtacgtcaagggtctggctgacggggctggagatcatgtgaccgcttttactctacatcagtattatttcgatggaaatacgagtgatgttagtacctacttggatgcgacgtactttaagaagttgcaacagttattcgataaggtaaaagacgtactcaagaattctccacataaggacaaacccttgtggctaggggaaacctcttccggctacaacagtgggactaaagatgtatccgatagatacgtgtcggggttcttgacgctggacaagttggggctttcggcggcaaataacgtcaaggtggtcatcagacaaacgatttataatggttactatggtttgcttgacaagaatactttggagcccaatccggactactggctgatgcacgtccacaattccttagttggtaataccgttttcaaggtcgatgtcagcgatcccacaaacaaagcccgtgtttacgctcagtgtacgaagaccaatagtaaacatacccagtcacgttattataaggggtccctaaccattttcgcgttgaatgtaggtgatgaagatgttacactcaagattgatcaatacagtggtaagaaaatatactcatatattctgacgcctgaaggcggccagttaacctctcaaaaggtactgcttaacggtaaagaattgaagttagtgtcagatcaacttccagaacttaacgcggacgaaagtaaaacatccttcacattgtctcccaaaacttttggattctttgtggtctcggatgccaacgttgaagcttgcaagaaataa

SEQ ID NO: 24 - DNA, 1740 bp, Hirudo nipponia
  "Reencoded nucleic acid sequence of hyaluronidase (HYAL) originating from Hirudo Nipponia with a N-terminal secretion signal and a C-terminal anchoring signal"
  Reencoded nucleic acid sequence of hyaluronidase (HYAL) originating from Hirudo Nipponia with a N-terminal secretion signal and a C-terminal anchoring signal
atgcaattctctactgtcgcttccgttgctttcgtcgctttggctaactttgttgccgctatgaaggagatagcagttaccatcgatgataagaatgttatagcgtctgtcagtgaaagcttccatggtgtggctttcgacgcaagcctattctcacctaaagggctatggtcgtttgttgacattacttcacccaagttattcaagcttctggagggactctcccctggttatttccgtgtcggcggcacatttgcgaactggttattcttcgacctcgatgaaaacaacaagtggaaggattactgggcttttaaggacaagactccagagaccgccacgattacccgacggtggctcttcaggaagcaaaacaacctcaagaaggaaacctttgatgatttggtaaagcttacaaaggggtccaagatgcggctgctatttgatctaaacgcagaggtccgtacaggatatgagataggcaagaagatgacatcaacttgggactcaagcgaggcagaaaagttgttcaaatattgcgttagcaagggatatggagataatatcgattgggagttaggcaacgaacctgatcacacgtcagcacacaatttgacagagaagcaagtaggtgaagattttaaggccctacacaaggtgttggaaaagtatccaacacttaataaaggtagcttggttggtccagacgttgggtggatgggagtgtcgtacgtcaagggtctggctgacggggctggagatcatgtgaccgcttttactctacatcagtattatttcgatggaaatacgagtgatgttagtacctacttggatgcgacgtactttaagaagttgcaacagttattcgataaggtaaaagacgtactcaagaattctccacataaggacaaacccttgtggctaggggaaacctcttccggctacaacagtgggactaaagatgtatccgatagatacgtgtcggggttcttgacgctggacaagttggggctttcggcggcaaataacgtcaaggtggtcatcagacaaacgatttataatggttactatggtttgcttgacaagaatactttggagcccaatccggactactggctgatgcacgtccacaattccttagttggtaataccgttttcaaggtcgatgtcagcgatcccacaaacaaagcccgtgtttacgctcagtgtacgaagaccaatagtaaacatacccagtcacgttattataaggggtccctaaccattttcgcgttgaatgtaggtgatgaagatgttacactcaagattgatcaatacagtggtaagaaaatatactcatatattctgacgcctgaaggcggccagttaacctctcaaaaggtactgcttaacggtaaagaattgaagttagtgtcagatcaacttccagaacttaacgcggacgaaagtaaaacatccttcacattgtctcccaaaacttttggattctttgtggtctcggatgccaacgttgaagcttgcaagaaaggatccgccatttctcaaatcactgacggtcaaatccaagctactaccactgctaccaccgaagctaccaccactgctgccccatcttccaccgttgaaactgtttctccatccagcaccgaaactatctctcaacaaactgaaaatggtgctgctaaggccgctgtcggtatgggtgccggtgctctagctgctgctgctatgttgttataa

SEQ ID NO: 25 - DNA, 1206 bp, Loxosceles intermedia
  "Reencoded nucleic acid sequence of hyaluronidase (HYAL) originating from Loxosceles intermedia with a N-terminal secretion signal"
  Reencoded nucleic acid sequence of hyaluronidase (HYAL) originating from Loxosceles intermedia with a N-terminal secretion signal
atgcagttttcaaccgttgcgagcgtcgcttttgtggctcttgctaatttcgttgccgccttcgatgtcttctggaatgttccgtcgcagcaatgcaagaaatatggtatgaaattcgttccgctcttagagcaatactctatcctagtcaacaaagaagacaatttcaagggcgacaaaataacgatcttttatgagtcacagctcgggctttacccacatattggtgcaaacgacgagtcgtttaatggcgggataccacaattaggtgacctgaaagcacacttagaaaagtcagcggttgatatacgacgtgatattttggataagtcggcgactggtctaagaattatagactgggaagcatggagaccaatatgggaattcaactggtctagcctacgaaagtaccaagataaaatgaagaaagtcgtccgccagtttaacccgactgctcatgaatccacagtggccaaactagcacataatgagtgggaaaatagtagtaagtcttggatgctttctacattgcagttgggtaagcaacttcgtccaaactctgtatggtgctattatttatttcccgactgttataactatgatggcaactcagtccaagaatttcagtgttctgaagctatccgtaaggggaacgataggttgaaatggttgtgggaagaatcgacagctgtatgcccatctatctacataaaagaaggccaactgaccaattataccttgcaaaagagaatctggtttaccaatgggagattacaggaagccttgagagtagctcaacctaaagcgcgtatttatccatacataaattactccatcaaacccggaatgatggtgcctgaagttgagttttggcggttaatcgctcagatagcctcgctgggtatggatggagcagtgatttggggatcaagtgcgagtgtaggcagtaagaatcattgtgcgcaattaatgaagtacattgcagacgtattgggtcctgcaactttgcgcataaaagaaaatgtagcacggtgcagtaaacaggcgtgctctggtaggggtagatgtacctggcctaaagatacctctgttattgcttggaagttcctcgttgaaaaggaagactatgacttttatctgggtgatatagagtgtaaatgtgttgaaggctacgaaggtaggtactgtgaacaaaagactaagtaa

SEQ ID NO: 26 - DNA, 1416 bp, Loxosceles intermedia
  "Reencoded nucleic acid sequence of hyaluronidase (HYAL) originating from Loxosceles intermedia with a N-terminal secretion signal and a C-terminal anchoring signal"
  Reencoded nucleic acid sequence of hyaluronidase (HYAL) originating from Loxosceles intermedia with a N-terminal secretion signal and a C-terminal anchoring signal
atgcagttttcaaccgttgcgagcgtcgcttttgtggctcttgctaatttcgttgccgccttcgatgtcttctggaatgttccgtcgcagcaatgcaagaaatatggtatgaaattcgttccgctcttagagcaatactctatcctagtcaacaaagaagacaatttcaagggcgacaaaataacgatcttttatgagtcacagctcgggctttacccacatattggtgcaaacgacgagtcgtttaatggcgggataccacaattaggtgacctgaaagcacacttagaaaagtcagcggttgatatacgacgtgatattttggataagtcggcgactggtctaagaattatagactgggaagcatggagaccaatatgggaattcaactggtctagcctacgaaagtaccaagataaaatgaagaaagtcgtccgccagtttaacccgactgctcatgaatccacagtggccaaactagcacataatgagtgggaaaatagtagtaagtcttggatgctttctacattgcagttgggtaagcaacttcgtccaaactctgtatggtgctattatttatttcccgactgttataactatgatggcaactcagtccaagaatttcagtgttctgaagctatccgtaaggggaacgataggttgaaatggttgtgggaagaatcgacagctgtatgcccatctatctacataaaagaaggccaactgaccaattataccttgcaaaagagaatctggtttaccaatgggagattacaggaagccttgagagtagctcaacctaaagcgcgtatttatccatacataaattactccatcaaacccggaatgatggtgcctgaagttgagttttggcggttaatcgctcagatagcctcgctgggtatggatggagcagtgatttggggatcaagtgcgagtgtaggcagtaagaatcattgtgcgcaattaatgaagtacattgcagacgtattgggtcctgcaactttgcgcataaaagaaaatgtagcacggtgcagtaaacaggcgtgctctggtaggggtagatgtacctggcctaaagatacctctgttattgcttggaagttcctcgttgaaaaggaagactatgacttttatctgggtgatatagagtgtaaatgtgttgaaggctacgaaggtaggtactgtgaacaaaagactaagggatccgccatttctcaaatcactgacggtcaaatccaagctactaccactgctaccaccgaagctaccaccactgctgccccatcttccaccgttgaaactgtttctccatccagcaccgaaactatctctcaacaaactgaaaatggtgctgctaaggccgctgtcggtatgggtgccggtgctctagctgctgctgctatgttgttataa

SEQ ID NO: 27 - DNA, 1218 bp, Tityus serrulatus
  "Reencoded nucleic acid sequence of hyaluronidase (HYAL) originating from Tityus serrulatus with a N-terminal secretion signal"
  Reencoded nucleic acid sequence of hyaluronidase (HYAL) originating from Tityus serrulatus with a N-terminal secretion signal
atgcaattctctactgtcgcttccgttgctttcgtcgctttggctaactttgttgccgctgctgattttaaagtttactgggaagtgccttccttcctttgttctaaacgttttaaaattaatgtaacggaagttttaacaagtcacgagattcttgtcaatcagggtgagagtttcaacggtgacaagatagtaatcttttacgaaaaccaattggggaagtacccgcatattgactcaaacaatgtggagatcaatggaggaatacttcaagtagccgatttggcgaagcatttgaaagtagccaaggataatatcactaaattcgtcccgaatcctaatttcaacggtgtcggagtgatcgactgggaagcttggcggccatcatgggaatttaactggggtaagttaaaagtatataaagaaaagagcattgacttggtcaagtcgaaacatccggagtggccctccgacagggttgaaaaggttgctaaagaggagtgggaggagagtgccaaagaatggatggtgaagaccctgaagttagcacaggaaatgcgaccgaacgcagtttggtgctattatctattccctgactgctacaattatttcggtaaggatcaaccctctcaattcagctgctcgtctcgaattcagaaggaaaattctcgtctttcttggctctggaatcaatcaacagccatttgcctaagcatttatatccaggaatcccatgttaccaaatataatatgtcccagcggacatggtggatcgatgcgagattaagagaagcaattcgagtcagcgaacacagaccaaacatacccatctacccttacattaattatattctacctggaactaatcaaactgtaccagcaatggactttaaaaggacactgggtcaaatagctagcctcggcctagatggtgctttgttatggggatctagctatcatgttttaacagaatctcaatgcaaaatcacttctgattatgtgaaatcagtgattgctcctaccgtggctactgtcgttctcaatacaaacagatgctcacagataatttgtaagggtcgcggcaactgtgtttggcctgaagaaccatttagttcttggaaatacttagttgaccccaaaatgccagtgttcaagccaaccaacatccactgtaaatgtaaaggttacctaggtagatactgtgagatcccaaagtaa

SEQ ID NO: 28 - DNA, 1428 bp, Tityus serrulatus
  "Reencoded nucleic acid sequence of hyaluronidase (HYAL) originating from Tityus serrulatus with a N-terminal secretion signal and a C-terminal anchoring signal"
  Reencoded nucleic acid sequence of hyaluronidase (HYAL) originating from Tityus serrulatus with a N-terminal secretion signal and a C-terminal anchoring signal
atgcaattctctactgtcgcttccgttgctttcgtcgctttggctaactttgttgccgctgctgattttaaagtttactgggaagtgccttccttcctttgttctaaacgttttaaaattaatgtaacggaagttttaacaagtcacgagattcttgtcaatcagggtgagagtttcaacggtgacaagatagtaatcttttacgaaaaccaattggggaagtacccgcatattgactcaaacaatgtggagatcaatggaggaatacttcaagtagccgatttggcgaagcatttgaaagtagccaaggataatatcactaaattcgtcccgaatcctaatttcaacggtgtcggagtgatcgactgggaagcttggcggccatcatgggaatttaactggggtaagttaaaagtatataaagaaaagagcattgacttggtcaagtcgaaacatccggagtggccctccgacagggttgaaaaggttgctaaagaggagtgggaggagagtgccaaagaatggatggtgaagaccctgaagttagcacaggaaatgcgaccgaacgcagtttggtgctattatctattccctgactgctacaattatttcggtaaggatcaaccctctcaattcagctgctcgtctcgaattcagaaggaaaattctcgtctttcttggctctggaatcaatcaacagccatttgcctaagcatttatatccaggaatcccatgttaccaaatataatatgtcccagcggacatggtggatcgatgcgagattaagagaagcaattcgagtcagcgaacacagaccaaacatacccatctacccttacattaattatattctacctggaactaatcaaactgtaccagcaatggactttaaaaggacactgggtcaaatagctagcctcggcctagatggtgctttgttatggggatctagctatcatgttttaacagaatctcaatgcaaaatcacttctgattatgtgaaatcagtgattgctcctaccgtggctactgtcgttctcaatacaaacagatgctcacagataatttgtaagggtcgcggcaactgtgtttggcctgaagaaccatttagttcttggaaatacttagttgaccccaaaatgccagtgttcaagccaaccaacatccactgtaaatgtaaaggttacctaggtagatactgtgagatcccaaagggatccgccatttctcaaatcactgacggtcaaatccaagctactaccactgctaccaccgaagctaccaccactgctgccccatcttccaccgttgaaactgtttctccatccagcaccgaaactatctctcaacaaactgaaaatggtgctgctaaggccgctgtcggtatgggtgccggtgctctagctgctgctgctatgttgttataa

SEQ ID NO: 29 - DNA, 1083 bp, Vespa magnifica
  "Reencoded nucleic acid sequence of hyaluronidase (HYAL) originating from Vespa magnifica with a N-terminal secretion signal"
  Reencoded nucleic acid sequence of hyaluronidase (HYAL) originating from Vespa magnifica with a N-terminal secretion signal
atgcaattttctacagtggcaagtgttgcattcgttgcactagccaactttgtggcggcagatagctgtgggtcaaactgcgaaaagagtgagagaccgaaaagggtcttcaacatttactggaacgtacctacattcatgtgtcaccagtacggactatactttgacgaggtcacgaattttaatataaagcacaacagcaaagacaattttcaaggggacaagatcgcgatcttttatgaccccggggagtttcccgctctgctgccactaaactatggtaagtacaagatcaggaatggtggtgttccacaagagggtaacatcaccatccatctgcagagattcatagagtacctagataagacctatccgaaccgtaacttttcaggcatcggtgtgatcgatttcgagaggtggagaccaattttcagacagaattggggtaatatgaagatttacaagaacttctccatcgatcttgtgcgtaaagagcatcctttctggaataagaaaatgatcgagttggaagcttctaaaagattcgagaaatacgcccgtctgttcatggaagaaacattaaagttggctaagaaaactagaaaacaggccgattggggctactacggttacccctattgcttcaacatgtctcctactaatttcgttcctgactgcgatgtcacagctagggatgagaacaacgagatgtcttggttgtttaacaaccagaatgtcctattaccaagtgtatacattaggagagagctaactcctgaccagaggattgggcttgtacaggggagagtgaaggaagctgtgagaatttcaaataaactgaagcactcacctaaagtcttcagctattggtggtatgtttaccaagacgagaccaacaccttcttaacggagaccgacgtcaagaagacgtttcaggagattgtgatcaacggtggagatgggattataatctggggttcgtcctctgatgtaaacagcttgtccaagtgtacgaggttaagggagtacctattgacagtcttgggaccaattgctgttaacgtgactgaagcagtaaactaa

SEQ ID NO: 30 - DNA, 1293 bp, Vespa magnifica
  "Reencoded nucleic acid sequence of hyaluronidase (HYAL) originating from Vespa magnifica with a N-terminal secretion signal and a C-terminal anchoring signal"
  Reencoded nucleic acid sequence of hyaluronidase (HYAL) originating from Vespa magnifica with a N-terminal secretion signal and a C-terminal anchoring signal
atgcaattttctacagtggcaagtgttgcattcgttgcactagccaactttgtggcggcagatagctgtgggtcaaactgcgaaaagagtgagagaccgaaaagggtcttcaacatttactggaacgtacctacattcatgtgtcaccagtacggactatactttgacgaggtcacgaattttaatataaagcacaacagcaaagacaattttcaaggggacaagatcgcgatcttttatgaccccggggagtttcccgctctgctgccactaaactatggtaagtacaagatcaggaatggtggtgttccacaagagggtaacatcaccatccatctgcagagattcatagagtacctagataagacctatccgaaccgtaacttttcaggcatcggtgtgatcgatttcgagaggtggagaccaattttcagacagaattggggtaatatgaagatttacaagaacttctccatcgatcttgtgcgtaaagagcatcctttctggaataagaaaatgatcgagttggaagcttctaaaagattcgagaaatacgcccgtctgttcatggaagaaacattaaagttggctaagaaaactagaaaacaggccgattggggctactacggttacccctattgcttcaacatgtctcctactaatttcgttcctgactgcgatgtcacagctagggatgagaacaacgagatgtcttggttgtttaacaaccagaatgtcctattaccaagtgtatacattaggagagagctaactcctgaccagaggattgggcttgtacaggggagagtgaaggaagctgtgagaatttcaaataaactgaagcactcacctaaagtcttcagctattggtggtatgtttaccaagacgagaccaacaccttcttaacggagaccgacgtcaagaagacgtttcaggagattgtgatcaacggtggagatgggattataatctggggttcgtcctctgatgtaaacagcttgtccaagtgtacgaggttaagggagtacctattgacagtcttgggaccaattgctgttaacgtgactgaagcagtaaacggatccgccatttctcaaatcactgacggtcaaatccaagctactaccactgctaccaccgaagctaccaccactgctgccccatcttccaccgttgaaactgtttctccatccagcaccgaaactatctctcaacaaactgaaaatggtgctgctaaggccgctgtcggtatgggtgccggtgctctagctgctgctgctatgttgttataa

SEQ ID NO: 31 - protein, 441 aa, Bothrops atrox
  Amino acid sequence of hyaluronidase (HYAL) originating from Bothrops atrox with a N-terminal secretion signal
  Amino acid sequence of hyaluronidase (HYAL) originating from Bothrops atrox with a N-terminal secretion signal
MQFSTVASVAFVALANFVAAPMYPNEPFLVFWNAPTTQCRLRYKVDLDLKTFHIVTNANDSLSGSAVTIFYPTHLGVYPHIDDRGHFFNGIIPQNESLVKHLNKSKSDINRMIPLRTFHGLGVIDWENWRPQWDRNWGSKNVYRNRSIQFARDLHPELSEDKIKRLAKQEFEKAAKSFMRDTLLLAEEMRPDGYWGYYLYPDCHNYNYKTKPDQYTGECPDIEMSRNNQLLWLWRDSTALFPNIYLETILRSSDNALKFVHHRLKEAMRIASMARNDYALPFFVYARPFYAYTFEPLTQEDLVTTVGETADMGAAGIVFWGSMQYASTVESCGKVKDYMNGPLGRYIVNVTTAAKICSRFLCKRHGRCVRKHSDSNAFLHLFPDSFRIMVHGNATEKKVIVKGKLELKNLIFLRNNFMCQCYQGWKGLYCEKHSIKEIRKI

SEQ ID NO: 32 - protein, 511 aa, Bothrops atrox
  Amino acid sequence of hyaluronidase (HYAL) originating from Bothrops atrox with a N-terminal secretion signal and a C-terminal anchoring signal
  Amino acid sequence of hyaluronidase (HYAL) originating from Bothrops atrox with a N-terminal secretion signal and a C-terminal anchoring signal
MQFSTVASVAFVALANFVAAPMYPNEPFLVFWNAPTTQCRLRYKVDLDLKTFHIVTNANDSLSGSAVTIFYPTHLGVYPHIDDRGHFFNGIIPQNESLVKHLNKSKSDINRMIPLRTFHGLGVIDWENWRPQWDRNWGSKNVYRNRSIQFARDLHPELSEDKIKRLAKQEFEKAAKSFMRDTLLLAEEMRPDGYWGYYLYPDCHNYNYKTKPDQYTGECPDIEMSRNNQLLWLWRDSTALFPNIYLETILRSSDNALKFVHHRLKEAMRIASMARNDYALPFFVYARPFYAYTFEPLTQEDLVTTVGETADMGAAGIVFWGSMQYASTVESCGKVKDYMNGPLGRYIVNVTTAAKICSRFLCKRHGRCVRKHSDSNAFLHLFPDSFRIMVHGNATEKKVIVKGKLELKNLIFLRNNFMCQCYQGWKGLYCEKHSIKEIRKIGSAISQITDGQIQATTTATTEATTTAAPSSTVETVSPSSTETISQQTENGAAKAAVGMGAGALAAAAMLL

SEQ ID NO: 33 - protein, 398 aa, Cupiennius salei
  Amino acid sequence of hyaluronidase (HYAL) originating from Cupiennius salei with a N-terminal secretion signal
  Amino acid sequence of hyaluronidase (HYAL) originating from Cupiennius salei with a N-terminal secretion signal
MQFSTVASVAFVALANFVAAFKIYWNVPTFQCTHNYKIDYVKLLSTYGIQVNDGGKFQGNQVTIFYETQLGLYPRILKSGKMENGGIPQRGNFEKHLEKASTDLQKVIPWKEFSGLGVIDWEAWRPTWEFNWEPLRIYQTESIKRAKELHPTANDSAVKEIAERQWEDSAKLYMLETLRLAKKLRPQAPWCYYLFPDCYNYVGKKPKDFQCSASIRKGNDKLSWLWKDSTALCPSIYVYESQLDRYSFEQRTWRDNEKLREALRVATRTSKIYPYVNYFDKELIPEQEVWRMLAQAAAVGGSGAVIWGSSAAVASEELCKSLKQYIIETLGPAAEKVAWRSDLCSKEICNNQGRCTFPDDDYANAWKLFTDDTVKFYAGNITCRCSENYSGRFCEKKN

SEQ ID NO: 34 - protein, 468 aa, Cupiennius salei
  Amino acid sequence of hyaluronidase (HYAL) originating from Cupiennius salei with a N-terminal secretion signal and a C-terminal anchoring signal
  Amino acid sequence of hyaluronidase (HYAL) originating from Cupiennius salei with a N-terminal secretion signal and a C-terminal anchoring signal
MQFSTVASVAFVALANFVAAFKIYWNVPTFQCTHNYKIDYVKLLSTYGIQVNDGGKFQGNQVTIFYETQLGLYPRILKSGKMENGGIPQRGNFEKHLEKASTDLQKVIPWKEFSGLGVIDWEAWRPTWEFNWEPLRIYQTESIKRAKELHPTANDSAVKEIAERQWEDSAKLYMLETLRLAKKLRPQAPWCYYLFPDCYNYVGKKPKDFQCSASIRKGNDKLSWLWKDSTALCPSIYVYESQLDRYSFEQRTWRDNEKLREALRVATRTSKIYPYVNYFDKELIPEQEVWRMLAQAAAVGGSGAVIWGSSAAVASEELCKSLKQYIIETLGPAAEKVAWRSDLCSKEICNNQGRCTFPDDDYANAWKLFTDDTVKFYAGNITCRCSENYSGRFCEKKNGSAISQITDGQIQATTTATTEATTTAAPSSTVETVSPSSTETISQQTENGAAKAAVGMGAGALAAAAMLL

SEQ ID NO: 35 - protein, 579 aa, Hirudo nipponia
  Amino acid sequence of hyaluronidase (HYAL) originating from Hirudo Nipponia with a N-terminal secretion signal
  Amino acid sequence of hyaluronidase (HYAL) originating from Hirudo Nipponia with a N-terminal secretion signal
MQFSTVASVAFVALANFVAAMKEIAVTIDDKNVIASVSESFHGVAFDASLFSPKGLWSFVDITSPKLFKLLEGLSPGYFRVGGTFANWLFFDLDENNKWKDYWAFKDKTPETATITRRWLFRKQNNLKKETFDDLVKLTKGSKMRLLFDLNAEVRTGYEIGKKMTSTWDSSEAEKLFKYCVSKGYGDNIDWELGNEPDHTSAHNLTEKQVGEDFKALHKVLEKYPTLNKGSLVGPDVGWMGVSYVKGLADGAGDHVTAFTLHQYYFDGNTSDVSTYLDATYFKKLQQLFDKVKDVLKNSPHKDKPLWLGETSSGYNSGTKDVSDRYVSGFLTLDKLGLSAANNVKVVIRQTIYNGYYGLLDKNTLEPNPDYWLMHVHNSLVGNTVFKVDVSDPTNKARVYAQCTKTNSKHTQSRYYKGSLTIFALNVGDEDVTLKIDQYSGKKIYSYILTPEGGQLTSQKVLLNGKELKLVSDQLPELNADESKTSFTLSPKTFGFFVVSDANVEACKKGSAISQITDGQIQATTTATTEATTTAAPSSTVETVSPSSTETISQQTENGAAKAAVGMGAGALAAAAMLL

SEQ ID NO: 36 - protein, 509 aa, Hirudo nipponia
  Amino acid sequence of hyaluronidase (HYAL) originating from Hirudo Nipponia with a N-terminal secretion signal and a C-terminal anchoring signal
  Amino acid sequence of hyaluronidase (HYAL) originating from Hirudo Nipponia with a N-terminal secretion signal and a C-terminal anchoring signal
MQFSTVASVAFVALANFVAAMKEIAVTIDDKNVIASVSESFHGVAFDASLFSPKGLWSFVDITSPKLFKLLEGLSPGYFRVGGTFANWLFFDLDENNKWKDYWAFKDKTPETATITRRWLFRKQNNLKKETFDDLVKLTKGSKMRLLFDLNAEVRTGYEIGKKMTSTWDSSEAEKLFKYCVSKGYGDNIDWELGNEPDHTSAHNLTEKQVGEDFKALHKVLEKYPTLNKGSLVGPDVGWMGVSYVKGLADGAGDHVTAFTLHQYYFDGNTSDVSTYLDATYFKKLQQLFDKVKDVLKNSPHKDKPLWLGETSSGYNSGTKDVSDRYVSGFLTLDKLGLSAANNVKVVIRQTIYNGYYGLLDKNTLEPNPDYWLMHVHNSLVGNTVFKVDVSDPTNKARVYAQCTKTNSKHTQSRYYKGSLTIFALNVGDEDVTLKIDQYSGKKIYSYILTPEGGQLTSQKVLLNGKELKLVSDQLPELNADESKTSFTLSPKTFGFFVVSDANVEACKK

SEQ ID NO: 37 - protein, 401 aa, Loxosceles intermedia
  Amino acid sequence of hyaluronidase (HYAL) originating from Loxosceles intermedia with a N-terminal secretion signal
  Amino acid sequence of hyaluronidase (HYAL) originating from Loxosceles intermedia with a N-terminal secretion signal
MQFSTVASVAFVALANFVAAFDVFWNVPSQQCKKYGMKFVPLLEQYSILVNKEDNFKGDKITIFYESQLGLYPHIGANDESFNGGIPQLGDLKAHLEKSAVDIRRDILDKSATGLRIIDWEAWRPIWEFNWSSLRKYQDKMKKVVRQFNPTAHESTVAKLAHNEWENSSKSWMLSTLQLGKQLRPNSVWCYYLFPDCYNYDGNSVQEFQCSEAIRKGNDRLKWLWEESTAVCPSIYIKEGQLTNYTLQKRIWFTNGRLQEALRVAQPKARIYPYINYSIKPGMMVPEVEFWRLIAQIASLGMDGAVIWGSSASVGSKNHCAQLMKYIADVLGPATLRIKENVARCSKQACSGRGRCTWPKDTSVIAWKFLVEKEDYDFYLGDIECKCVEGYEGRYCEQKTK

SEQ ID NO: 38 - protein, 471 aa, Loxosceles intermedia
  Amino acid sequence of hyaluronidase (HYAL) originating from Loxosceles intermedia with a N-terminal secretion signal and a C-terminal anchoring signal
  Amino acid sequence of hyaluronidase (HYAL) originating from Loxosceles intermedia with a N-terminal secretion signal and a C-terminal anchoring signal
MQFSTVASVAFVALANFVAAFDVFWNVPSQQCKKYGMKFVPLLEQYSILVNKEDNFKGDKITIFYESQLGLYPHIGANDESFNGGIPQLGDLKAHLEKSAVDIRRDILDKSATGLRIIDWEAWRPIWEFNWSSLRKYQDKMKKVVRQFNPTAHESTVAKLAHNEWENSSKSWMLSTLQLGKQLRPNSVWCYYLFPDCYNYDGNSVQEFQCSEAIRKGNDRLKWLWEESTAVCPSIYIKEGQLTNYTLQKRIWFTNGRLQEALRVAQPKARIYPYINYSIKPGMMVPEVEFWRLIAQIASLGMDGAVIWGSSASVGSKNHCAQLMKYIADVLGPATLRIKENVARCSKQACSGRGRCTWPKDTSVIAWKFLVEKEDYDFYLGDIECKCVEGYEGRYCEQKTKGSAISQITDGQIQATTTATTEATTTAAPSSTVETVSPSSTETISQQTENGAAKAAVGMGAGALAAAAMLL

SEQ ID NO: 39 - protein, 405 aa, Tityus serrulatus
  Amino acid sequence of hyaluronidase (HYAL) originating from Tityus serrulatus with a N-terminal secretion signal
  Amino acid sequence of hyaluronidase (HYAL) originating from Tityus serrulatus with a N-terminal secretion signal
MQFSTVASVAFVALANFVAAADFKVYWEVPSFLCSKRFKINVTEVLTSHEILVNQGESFNGDKIVIFYENQLGKYPHIDSNNVEINGGILQVADLAKHLKVAKDNITKFVPNPNFNGVGVIDWEAWRPSWEFNWGKLKVYKEKSIDLVKSKHPEWPSDRVEKVAKEEWEESAKEWMVKTLKLAQEMRPNAVWCYYLFPDCYNYFGKDQPSQFSCSSRIQKENSRLSWLWNQSTAICLSIYIQESHVTKYNMSQRTWWIDARLREAIRVSEHRPNIPIYPYINYILPGTNQTVPAMDFKRTLGQIASLGLDGALLWGSSYHVLTESQCKITSDYVKSVIAPTVATVVLNTNRCSQIICKGRGNCVWPEEPFSSWKYLVDPKMPVFKPTNIHCKCKGYLGRYCEIPK

SEQ ID NO: 40 - protein, 475 aa, Tityus serrulatus
  Amino acid sequence of hyaluronidase (HYAL) originating from Tityus serrulatus with a N-terminal secretion signal and a C-terminal anchoring signal
  Amino acid sequence of hyaluronidase (HYAL) originating from Tityus serrulatus with a N-terminal secretion signal and a C-terminal anchoring signal
MQFSTVASVAFVALANFVAAADFKVYWEVPSFLCSKRFKINVTEVLTSHEILVNQGESFNGDKIVIFYENQLGKYPHIDSNNVEINGGILQVADLAKHLKVAKDNITKFVPNPNFNGVGVIDWEAWRPSWEFNWGKLKVYKEKSIDLVKSKHPEWPSDRVEKVAKEEWEESAKEWMVKTLKLAQEMRPNAVWCYYLFPDCYNYFGKDQPSQFSCSSRIQKENSRLSWLWNQSTAICLSIYIQESHVTKYNMSQRTWWIDARLREAIRVSEHRPNIPIYPYINYILPGTNQTVPAMDFKRTLGQIASLGLDGALLWGSSYHVLTESQCKITSDYVKSVIAPTVATVVLNTNRCSQIICKGRGNCVWPEEPFSSWKYLVDPKMPVFKPTNIHCKCKGYLGRYCEIPKGSAISQITDGQIQATTTATTEATTTAAPSSTVETVSPSSTETISQQTENGAAKAAVGMGAGALAAAAMLL

SEQ ID NO: 41 - protein, 360 aa, Vespa magnifica
  Amino acid sequence of hyaluronidase (HYAL) originating from Vespa magnifica with a N-terminal secretion signal
  Amino acid sequence of hyaluronidase (HYAL) originating from Vespa magnifica with a N-terminal secretion signal
MQFSTVASVAFVALANFVAADSCGSNCEKSERPKRVFNIYWNVPTFMCHQYGLYFDEVTNFNIKHNSKDNFQGDKIAIFYDPGEFPALLPLNYGKYKIRNGGVPQEGNITIHLQRFIEYLDKTYPNRNFSGIGVIDFERWRPIFRQNWGNMKIYKNFSIDLVRKEHPFWNKKMIELEASKRFEKYARLFMEETLKLAKKTRKQADWGYYGYPYCFNMSPTNFVPDCDVTARDENNEMSWLFNNQNVLLPSVYIRRELTPDQRIGLVQGRVKEAVRISNKLKHSPKVFSYWWYVYQDETNTFLTETDVKKTFQEIVINGGDGIIIWGSSSDVNSLSKCTRLREYLLTVLGPIAVNVTEAVN

SEQ ID NO: 42 - protein, 428 aa, Vespa magnifica
  Amino acid sequence of hyaluronidase (HYAL) originating from Vespa magnifica with a N-terminal secretion signal and a C-terminal anchoring signal
  Amino acid sequence of hyaluronidase (HYAL) originating from Vespa magnifica with a N-terminal secretion signal and a C-terminal anchoring signal
MQFSTVASVAFVALANFVAADSCGSNCEKSERPKRVFNIYWNVPTFMCHQYGLYFDEVTNFNIKHNSKDNFQGDKIAIFYDPGEFPALLPLNYGKYKIRNGGVPQEGNITIHLQRFIEYLDKTYPNRNFSGIGVIDFERWRPIFRQNWGNMKIYKNFSIDLVRKEHPFWNKKMIELEASKRFEKYARLFMEETLKLAKKTRKQADWGYYGYPYCFNMSPTNFVPDCDVTARDENNEMSWLFNNQNVLLPSVYIRRELTPDQRIGLVQGRVKEAVRISNKLKHSPKVFSYWWYVYQDETNTFLTETDVKKTFQEIVINGGDGIIIWGSSSDVNSLSKCTRLREYLLTVLGPIAVNVTEAVNAISQITDGQIQATTTATTEATTTAAPSSTVETVSPSSTETISQQTENGAAKAAVGMGAGALAAAAMLL

SEQ ID NO: 43 - DNA, 60 bp, Artificial Sequence
  "Nucleic acid sequence of the secretion sequence added in 5â  "
  Nucleic acid sequence of the secretion sequence added in 5â
atgcaatttagcacagtcgcatcagtagccttcgttgccttggccaacttcgtggcagca

SEQ ID NO: 44 - protein, 20 aa, Artificial Sequence
  Amino acid sequence of the secretion sequence added in N-ter
  Amino acid sequence of the secretion sequence added in N-ter
MQFSTVASVAFVALANFVAA

SEQ ID NO: 45 - DNA, 213 bp, Artificial Sequence
  "Nucleic acid sequence of the anchoring sequence added in 3â  "
  Nucleic acid sequence of the anchoring sequence added in 3â
ggatccgccatttctcaaatcactgacggtcaaatccaagctactaccactgctaccaccgaagctaccaccactgctgccccatcttccaccgttgaaactgtttctccatccagcaccgaaactatctctcaacaaactgaaaatggtgctgctaaggccgctgtcggtatgggtgccggtgctctagctgctgctgctatgttgttataa

SEQ ID NO: 46 - protein, 68 aa, Artificial Sequence
  Amino acid sequence of the anchoring sequence added in C-ter
  Amino acid sequence of the anchoring sequence added in C-ter
AISQITDGQIQATTTATTEATTTAAPSSTVETVSPSSTETISQQTENGAAKAAVGMGAGALAAAAMLL

SEQ ID NO: 47 - DNA, 2154 bp, Saccharomyces cerevisiae
  "Nucleic acid sequence of glutamine-fructose-6-phosphate amidotransferase (GFA1) originating from"
  Nucleic acid sequence of glutamine-fructose-6-phosphate amidotransferase (GFA1) originating from
atgtgtggtatctttggttactgcaattatctagtggaaagatccagaggagaaattatcgacaccttagtggatggtttacaaagattagaatatagaggctatgattccaccggtattgctatcgatggtgacgaagctgattctactttcatctataagcaaatcggtaaagtgagtgctttgaaagaggagattactaagcaaaatccgaacagagacgttacttttgtctctcattgtggtattgcgcatactagatgggctactcacggtcgaccagaacaagttaactgtcaccctcaaagatctgacccagaagaccaatttgtggtcgttcataatggtatcatcacaaattttagagaactgaagactcttttaattaacaaaggttataaattcgaaagtgataccgataccgagtgtattgctaaactatatttgcatttatacaatacaaatttacaaaatgggcatgacttagatttccacgaattaaccaagctagttcttttagaactagaaggttcatacgggttattatgtaaatcttgtcactatcctaatgaggttatcgccactagaaaagggtcccctttactgattggtgtcaaatctgaaaaaaaactaaaagtcgacttcgtggatgtggaatttcccgaagaaaacgctggtcaaccggaaattccattgaaatctaacaacaaatcatttggcttgggcccaaagaaagctcgtgaatttgaagctggttcccaaaatgccaatttactaccaattgccgccaatgaatttaacttgagacattctcaatccagggctttcctatcagaagatggatctccaacaccggtggaattttttgtttcttcggatgcggcatctgttgttaaacataccaagaaggtgctatttttagaagatgacgatttggctcatatttacgatggtgagttacatattcatagatctagaagagaagtaggcgcatcaatgacaaggtccattcaaactttagagatggagttagctcagatcatgaagggcccttacgaccattttatgcaaaaggaaatctatgagcaaccagaatctactttcaatactatgagaggtagaatcgactatgaaaataataaagtgatattgggtggtttaaaggcatggttaccagttgtcagaagagcacggagactgatcatgatcgcatgcggtacttcttatcattcatgtttggctactcgtgctatcttcgaagaattatcagatatcccagttagtgtggaattagcgtctgactttctggacagaaaatgccctgtcttcagagacgatgtatgcgtgtttgtttcacaaagtggtgaaactgcggataccatgctggctctaaattattgtttagaaagaggagccttaactgtcggaattgttaacagtgttggttcttctatctctcgtgtcacccactgtggtgttcatattaacgctggtcctgaaattggtgttgcctctacaaaagcttatacttcccagtatattgccttagtgatgtttgctctatcgctgtcagatgaccgtgtatcgaaaatagacagaagaattgaaatcattcaaggcttgaagttaatcccgggccaaattaagcaggtattaaagctggaaccaagaataaaaaagctctgtgcgactgaattaaaggatcaaaaatctctattgttattgggtagaggttaccaatttgctgctgctctggaaggtgctttgaagatcaaagaaatttcttatatgcattctgaaggtgttttggcaggtgagttgaagcacggtgtcttggccttggtggacgaaaacttgccaatcattgcttttggtaccagagactctctattccctaaagtagtttcctctattgagcaagttactgtaagaaagggccatccaattattatttgtaacgaaaatgatgaagtgtgggcgcaaaaatctaaatcaatcgacctgcaaaccttagaagttccacaaactgttgattgtttacaaggtctaattaatattattccattacaactaatgtcatattggttggctgttaataaagggattgatgttgattttccaagaaacttggctaaatctgttaccgtcgaataa

SEQ ID NO: 48 - DNA, 1788 bp, Paramecium bursaria Chlorella virus 1
  "Reencoded nucleic acid sequence of glutamine-fructose-6-phosphate amidotransferase (GFA1) originating from Chlorella virus 1 (PBCV-1)"
  Reencoded nucleic acid sequence of glutamine-fructose-6-phosphate amidotransferase (GFA1) originating from Chlorella virus 1 (PBCV-1)
atgtgcgggatcttcggtgctgtgtcgaacaataatagcatagaagtttccatcaagggtatacagaagctagagtaccgcgggtacgattcgtgtggaatagcctatacagacggaggcgccattgaacggatcaggtcaatagatgggatcgacgacttaaggaagaaaacaataacagagtcttccccggtagctatcgctcattcaaggtggagtaccactgggattccaagtgttgtgaacgcccacccgcacatctctcggggcacgtctggatgcgagtcgcgcattgcagtcgtacacaatggcattattgaaaattaccagcagatccgcaagtacttgataaatcttgggtatactttcgattcacagaccgacacggaagtcattgctcatctaatagactcgcagtataacgggaacatcctgcacaccgtccaaatggcagttaagcacctcaaaggaagctacgccatagcagtcatgtgccataaggagtccgggaagatcgtggtggcaaaacagaagagtccgttggtattgggtataggaagcgacggagcttattatatcgcatcggacgtattggctcttcccactaacaaagtggtctacataagtgacggattctctgctgagttaagtcctggatcgatgactatctatgatctggatggcaataaggtagaatacgaggtggaagacgttgaaatggagcagacgtcgatgtctttagataactttgatcactacatgatcaaagagatcaatgaacagccgatatcaattctcaatactattaagaacaaaggattctatgcagagatatttggtgatctagcacatgaaatatttcagaagatcgacaatatattgattctagcctgcggaacttcgtatcatgcaggtctcgtcgggaagcaatggatagagaccatctcacgcatcccggtggatgttcatattgcaagcgagtatgagccgacaattccacgagccaatacacttgtgataacgattagtcaaagcggcgagactgcggatacaatcgcagcccttcaacgagcgcaaaacgcaggaatgatatacactttgtgtatctgcaacagccccaagtcaactctagtgcgcgagtcgataatgaaatacataaccaaatgcggttcagaagtttctgttgccagtactaaagcatttacgtcgcaacttgtggtgttgtatatgcttgcgaacgttcttgcgaacaaaactgatgatctgctaggggatcttcctcaagctatcgagagagtaatctgtcttactaatgacgaaatgaagcgttgggcggatgaaatttgtactgccaaaagtgccatcttcttagggagaggactgaacgcacctgtagcatttgagggcgcgctaaagttgaaggaaatctcatatatccatgccgagggtttcctcggtggagagttgaagcatgggccgctggctttgttggacgataagatccctgtaatcgtgactgttgctgaccacgcttatttggatcacattaaggctaacatcgacgaggtattggcacgaaacgttaccgtatacgcgatcgtcgatcagtatgttaatattgaaccacaggagcgactgcatgtagtaaaagtgccgtttgtgagtaaagagttttctcccatcatccacacaattccgatgcaattgttatcgtattatgtcgcgatcaagctgggcaagaacgttgacaagccacgtaacctggcgaaaagtgttacaacattctaa

SEQ ID NO: 49 - DNA, 1788 bp, Paramecium bursaria Chlorella virus 1
  "Reencoded nucleic acid sequence of glutamine-fructose-6-phosphate amidotransferase (GFA1) originating from Chlorella virus 1 (PBCV-1)"
  Reencoded nucleic acid sequence of glutamine-fructose-6-phosphate amidotransferase (GFA1) originating from Chlorella virus 1 (PBCV-1)
atgtgtggcatctttggagcagtgtcaaacaacaactctatcgaggtgtcaatcaagggtattcagaagctagaatatcgtgggtatgattcgtgcggtattgcgtatacagatgggggtgcgattgagcgtatacgttctattgacggcattgacgatctgcgtaagaaaacaatcacagaatcatcaccagtggccattgctcactcgcggtggagcaccactggaattccatcagtggtgaacgcacatcctcatatttctcgcggaaccagtgggtgtgagtctcgtatcgcggtagtccacaacggtatcattgaaaactatcagcagatccgaaaatatctcatcaatcttggttatacgtttgatagtcaaacggacacagaggtcattgcgcatttgattgattctcagtacaatgggaatatcttgcacaccgtccaaatggctgtcaagcacctgaagggctcttatgccattgcagttatgtgtcataaagagtctggtaaaatagtcgtggcgaaacagaagtcacccctcgtacttggaatcggctcagatggtgcttactacatcgcttcggacgtgctggcgctgccgacaaataaagttgtttatatttcagacggtttctccgcagaactatctccagggagtatgaccatttacgatcttgatggaaataaagtagaatatgaagtagaggacgttgaaatggaacaaactagtatgtctctcgataactttgatcattacatgattaaggaaattaatgagcaaccaatcagtattctaaacactataaaaaataaagggttctatgcagaaatattcggtgatttggctcatgaaatcttccaaaaaatagacaacatcctgatactggcttgtggtacaagttatcacgccggtcttgtaggaaaacagtggatagagaccatctctagaatccccgtggatgttcacatcgcgagtgaatacgaacctactattccgagagcgaacacattggtaatcactatttcacagtcgggtgaaactgcggacacgatagcggctttgcaacgggcccaaaacgccgggatgatttatacattgtgtatttgcaattcaccaaagagcactcttgttcgtgagagcattatgaagtacatcacgaaatgtggttctgaggtgtcagtggcatcaacgaaggcgtttacttctcagctcgtagtactgtacatgctggcaaacgtattggcaaataaaaccgatgatttgctgggagacctcccacaggcaatagaacgggtaatttgtttgacaaatgacgaaatgaaacgatgggccgacgaaatttgcactgcgaaatccgcgatcttcctgggaagaggactaaacgcaccagttgcctttgagggagcgttgaagctcaaagaaatctcttacattcatgcagagggcttcctgggaggtgagttgaaacacggccccctcgcactccttgatgacaagattcctgttatcgtaaccgtagcagatcatgcttatttggaccatatcaaagcaaatatcgacgaagtgcttgcgaggaacgttacggtatacgccatagtagaccagtatgtgaacatcgagccccaggaacgccttcacgtcgtcaaggttccgtttgtatccaaagaattttctccgataattcacactatcccgatgcaactgctttcgtattacgtggcaattaagcttggaaagaacgttgacaaaccaaggaatcttgcaaaatccgtgactaccttttaa

SEQ ID NO: 50 - protein, 717 aa, Saccharomyces cerevisiae
  Amino acid sequence of glutamine-fructose-6-phosphate amidotransferase (GFA1) originating from Saccharomyces cerevisiae
  Amino acid sequence of glutamine-fructose-6-phosphate amidotransferase (GFA1) originating from Saccharomyces cerevisiae
MCGIFGYCNYLVERSRGEIIDTLVDGLQRLEYRGYDSTGIAIDGDEADSTFIYKQIGKVSALKEEITKQNPNRDVTFVSHCGIAHTRWATHGRPEQVNCHPQRSDPEDQFVVVHNGIITNFRELKTLLINKGYKFESDTDTECIAKLYLHLYNTNLQNGHDLDFHELTKLVLLELEGSYGLLCKSCHYPNEVIATRKGSPLLIGVKSEKKLKVDFVDVEFPEENAGQPEIPLKSNNKSFGLGPKKAREFEAGSQNANLLPIAANEFNLRHSQSRAFLSEDGSPTPVEFFVSSDAASVVKHTKKVLFLEDDDLAHIYDGELHIHRSRREVGASMTRSIQTLEMELAQIMKGPYDHFMQKEIYEQPESTFNTMRGRIDYENNKVILGGLKAWLPVVRRARRLIMIACGTSYHSCLATRAIFEELSDIPVSVELASDFLDRKCPVFRDDVCVFVSQSGETADTMLALNYCLERGALTVGIVNSVGSSISRVTHCGVHINAGPEIGVASTKAYTSQYIALVMFALSLSDDRVSKIDRRIEIIQGLKLIPGQIKQVLKLEPRIKKLCATELKDQKSLLLLGRGYQFAAALEGALKIKEISYMHSEGVLAGELKHGVLALVDENLPIIAFGTRDSLFPKVVSSIEQVTARKGHPIIICNENDEVWAQKSKSIDLQTLEVPQTVDCLQGLINIIPLQLMSYWLAVNKGIDVDFPRNLAKSVTVE

SEQ ID NO: 51 - protein, 595 aa, Paramecium bursaria Chlorella virus 1
  Amino acid sequence of glutamine-fructose-6-phosphate amidotransferase (GFA1) originating from Chlorella virus 1 (PBCV-1)
  Amino acid sequence of glutamine-fructose-6-phosphate amidotransferase (GFA1) originating from Chlorella virus 1 (PBCV-1)
MCGIFGAVSNNNSIEVSIKGIQKLEYRGYDSCGIAYTDGGAIERIRSIDGIDDLRKKTITESSPVAIAHSRWSTTGIPSVVNAHPHISRGTSGCESRIAVVHNGIIENYQQIRKYLINLGYTFDSQTDTEVIAHLIDSQYNGNILHTVQMAVKHLKGSYAIAVMCHKESGKIVVAKQKSPLVLGIGSDGAYYIASDVLALPTNKVVYISDGFSAELSPGSMTIYDLDGNKVEYEVEDVEMEQTSMSLDNFDHYMIKEINEQPISILNTIKNKGFYAEIFGDLAHEIFQKIDNILILACGTSYHAGLVGKQWIETISRIPVDVHIASEYEPTIPRANTLVITISQSGETADTIAALQRAQNAGMIYTLCICNSPKSTLVRESIMKYITKCGSEVSVASTKAFTSQLVVLYMLANVLANKTDDLLGDLPQAIERVICLTNDEMKRWADEICTAKSAIFLGRGLNAPVAFEGALKLKEISYIHAEGFLGGELKHGPLALLDDKIPVIVTVADHAYLDHIKANIDEVLARNVTVYAIVDQYVNIEPQERLHVVKVPFVSKEFSPIIHTIPMQLLSYYVAIKLGKNVDKPRNLAKSVTTF

SEQ ID NO: 52 - DNA, 1434 bp, Saccharomyces cerevisiae
  "Nucleic acid sequence of UDP-N-acetylglucosamine pyrophosphorylase (QRI1) originating from Saccharomyces cerevisiae"
  Nucleic acid sequence of UDP-N-acetylglucosamine pyrophosphorylase (QRI1) originating from Saccharomyces cerevisiae
atgactgacacaaaacagctattcattgaagccggacaaagtcaacttttccacaattgggaaagcttgtctcgcaaagaccaagaagaattgctttcaaacctggagcaaatatcttccaagaggtcccctgcaaaactactggaagactgtcaaaatgctattaaattctcactagctaactcttctaaggatactggcgtcgaaatttcaccattgccccctacttcgtacgagtcgcttattggcaacagtaagaaagaaaatgaatactggcgtttaggccttgaagctattggcaagggtgaagtcgcagtgattttaatggctggcggacaaggtacgcggttaggatcctctcaaccaaagggctgttacgacattggattgccttctaagaaatctctttttcaaattcaagctgaaaagttgatcaggttgcaagatatggtaaaggacaaaaaggtagaaattccttggtatattatgacatcaggccccactagagcggctactgaggcatactttcaagaacacaattattttggcttgaataaagaacaaattacgttcttcaaccagggaaccctgcctgcctttgatttaaccgggaagcatttcctaatgaaagacccagtaaacctatctcaatcaccagatggaaatggtggactctaccgtgccatcaaggaaaacaagttgaacgaagactttgataggagaggaatcaagcatgtttacatgtactgtgtcgataatgtcctatctaaaatcgcagaccctgtatttattggttttgccatcaagcatggcttcgaactggccaccaaagccgttagaaagagagatgcgcatgaatcagttgggttaattgctactaaaaacgagaaaccatgtgtcatagaatattctgaaatttccaatgaattggctgaagcaaaggataaagatggcttattaaaactacgcgcaggcaacattgtaaatcattattacctagtggatttactaaaacgtgatttggatcagtggtgtgagaatatgccatatcacattgcgaagaagaaaattccagcttatgatagtgttaccggcaagtacactaagcctaccgaaccaaacggtataaaattagagcaattcatatttgatgtctttgacactgtaccactgaacaagtttgggtgcttagaagtagatagatgcaaagaattttcacctttaaaaaacggtcctggttctaagaacgataatcctgagaccagcagactagcatatttgaaactaggaacctcgtggttggaagatgcaggcgctattgtaaaagatggggtactagtcgaagtttccagcaaattgagttatgcaggtgaaaatctatcccagttcaaaggtaaagtctttgacagaagtggtatagtattagaaaaataa

SEQ ID NO: 53 - protein, 477 aa, Saccharomyces cerevisiae
  Amino acid sequence of UDP-N-acetylglucosamine pyrophosphorylase (QRI1) originating from Saccharomyces cerevisiae
  Amino acid sequence of UDP-N-acetylglucosamine pyrophosphorylase (QRI1) originating from Saccharomyces cerevisiae
MTDTKQLFIEAGQSQLFHNWESLSRKDQEELLSNLEQISSKRSPAKLLEDCQNAIKFSLANSSKDTGVEISPLPPTSYESLIGNSKKENEYWRLGLEAIGKGEVAVILMAGGQGTRLGSSQPKGCYDIGLPSKKSLFQIQAEKLIRLQDMVKDKKVEIPWYIMTSGPTRAATEAYFQEHNYFGLNKEQITFFNQGTLPAFDLTGKHFLMKDPVNLSQSPDGNGGLYRAIKENKLNEDFDRRGIKHVYMYCVDNVLSKIADPVFIGFAIKHGFELATKAVRKRDAHESVGLIATKNEKPCVIEYSEISNELAEAKDKDGLLKLRAGNIVNHYYLVDLLKRDLDQWCENMPYHIAKKKIPAYDSVTGKYTKPTEPNGIKLEQFIFDVFDTVPLNKFGCLEVDRCKEFSPLKNGPGSKNDNPETSRLAYLKLGTSWLEDAGAIVKDGVLVEVSSKLSYAGENLSQFKGKVFDRSGIVLEK

SEQ ID NO: 54 - DNA, 1713 bp, Saccharomyces cerevisiae
  "Nucleic acid sequence of Phosphoglucomutase-1 (PGM1) originating from Saccharomyces cerevisiae"
  Nucleic acid sequence of Phosphoglucomutase-1 (PGM1) originating from Saccharomyces cerevisiae
atgtcacttctaatagattctgtaccaacagttgcttataaggaccaaaaaccgggtacttcaggtttacgtaagaagaccaaggttttcatggatgagcctcattatactgagaacttcattcaagcaacaatgcaatctatccctaatggctcagagggaaccactttagttgttggaggagatggtcgtttctacaacgatgttatcatgaacaagattgccgcagtaggtgctgcaaacggtgtcagaaagttagtcattggtcaaggcggtttactttcaacaccagctgcttctcatataattagaacatacgaggaaaagtgtaccggtggtggtatcatattaactgcctcacacaacccaggcggtccagagaatgatttaggtatcaagtataatttacctaatggtgggccagctccagagagtgtcactaacgctatctgggaagcgtctaaaaaattaactcactataaaattataaagaacttccccaagttgaatttgaacaagcttggtaaaaaccaaaaatatggcccattgttagtggacataattgatcctgccaaagcatacgttcaatttctgaaggaaatttttgattttgacttaattaaaagcttcttagcgaaacagcgcaaagacaaagggtggaagttgttgtttgactccttaaatggtattacaggaccatatggtaaggctatatttgttgatgaatttggtttaccggcagaggaagttcttcaaaattggcaccctttacctgatttcggcggtttacatcccgatccgaatctaacctatgcacgaactcttgttgacagggttgaccgcgaaaaaattgcctttggagcagcctccgatggtgatggtgataggaatatgatttacggttatggccctgctttcgtttcgccaggtgattctgttgccattattgccgaatatgcacccgaaattccatacttcgccaaacaaggtatttatggcttggcacgttcatttcctacatcctcagccattgatcgtgttgcagcaaaaaagggattaagatgttacgaagttccaaccggctggaaattcttctgtgccttatttgatgctaaaaagctatcaatctgtggtgaagaatccttcggtacaggttccaatcatatcagagaaaaggacggtctatgggccattattgcttggttaaatatcttggctatctaccataggcgtaaccctgaaaaggaagcttcgatcaaaactattcaggacgaattttggaacgagtatggccgtactttcttcacaagatacgattacgaacatatcgaatgcgagcaggccgaaaaagttgtagctcttttgagtgaatttgtatcaaggccaaacgtttgtggctcccacttcccagctgatgagtctttaaccgttatcgattgtggtgatttttcgtatagagatctagatggctccatctctgaaaatcaaggccttttcgtaaagttttcgaatgggactaaatttgttttgaggttatccggcacaggcagttctggtgcaacaataagattatacgtagaaaagtatactgataaaaaggagaactatggccaaacagctgacgtcttcttgaaacccgtcatcaactccattgtaaaattcttaagatttaaagaaattttaggaacagacgaaccaacagtccgcacatag

SEQ ID NO: 55 - protein, 570 aa, Saccharomyces cerevisiae
  Amino acid sequence Phosphoglucomutase-1 (PGM1) originating from Saccharomyces cerevisiae
  Amino acid sequence Phosphoglucomutase-1 (PGM1) originating from Saccharomyces cerevisiae
MSLLIDSVPTVAYKDQKPGTSGLRKKTKVFMDEPHYTENFIQATMQSIPNGSEGTTLVVGGDGRFYNDVIMNKIAAVGAANGVRKLVIGQGGLLSTPAASHIIRTYEEKCTGGGIILTASHNPGGPENDLGIKYNLPNGGPAPESVTNAIWEASKKLTHYKIIKNFPKLNLNKLGKNQKYGPLLVDIIDPAKAYVQFLKEIFDFDLIKSFLAKQRKDKGWKLLFDSLNGITGPYGKAIFVDEFGLPAEEVLQNWHPLPDFGGLHPDPNLTYARTLVDRVDREKIAFGAASDGDGDRNMIYGYGPAFVSPGDSVAIIAEYAPEIPYFAKQGIYGLARSFPTSSAIDRVAAKKGLRCYEVPTGWKFFCALFDAKKLSICGEESFGTGSNHIREKDGLWAIIAWLNILAIYHRRNPEKEASIKTIQDEFWNEYGRTFFTRYDYEHIECEQAEKVVALLSEFVSRPNVCGSHFPADESLTVIDCGDFSYRDLDGSISENQGLFVKFSNGTKFVLRLSGTGSSGATIRLYVEKYTDKKENYGQTADVFLKPVINSIVKFLRFKEILGTDEPTVRT

SEQ ID NO: 56 - DNA, 1500 bp, Saccharomyces cerevisiae
  "Nucleic acid sequence of UTP--glucose-1-phosphate uridylyltransferase (UGP1) originating from"
  Nucleic acid sequence of UTP--glucose-1-phosphate uridylyltransferase (UGP1) originating from
atgtccactaagaagcacaccaaaacacattccacttatgcattcgagagcaacacaaacagcgttgctgcctcacaaatgagaaacgccttaaacaagttggcggactctagtaaacttgacgatgctgctcgcgctaagtttgagaacgaactggattcgtttttcacgcttttcaggagatatttggtagagaagtcttctagaaccaccttggaatgggacaagatcaagtctcccaacccggatgaagtggttaagtatgaaattatttctcagcagcccgagaatgtctcaaacctttccaaattggctgttttgaagttgaacggtgggctgggtacctccatgggctgcgttggccctaaatctgttattgaagtgagagagggaaacacctttttggatttgtctgttcgtcaaattgaatacttgaacagacagtacgatagcgacgtgccattgttattgatgaattctttcaacactgacaaggatacggaacacttgattaagaagtattccgctaacagaatcagaatcagatctttcaatcaatccaggttcccaagagtctacaaggattctttattgcctgtccccaccgaatacgattctccactggatgcttggtatccaccaggtcacggtgatttgtttgaatctttacacgtatctggtgaactggatgccttaattgcccaaggaagagaaatattatttgtttctaacggtgacaacttgggtgctaccgtcgacttaaaaattttaaaccacatgatcgagactggtgccgaatatataatggaattgactgataagaccagagccgatgttaaaggtggtactttgatttcttacgatggtcaagtccgtttattggaagtcgcccaagttccaaaagaacacattgacgaattcaaaaatatcagaaagtttaccaacttcaacacgaataacttatggatcaatctgaaagcagtaaagaggttgatcgaatcgagcaatttggagatggaaatcattccaaaccaaaaaactataacaagagacggtcatgaaattaatgtcttacaattagaaaccgcttgtggtgctgctatcaggcattttgatggtgctcacggtgttgtcgttccaagatcaagattcttgcctgtcaagacctgttccgatttgttgctggttaaatcagatctattccgtctggaacacggttctttgaagttagacccatcccgttttggtccaaacccattaatcaagttgggctcgcatttcaaaaaggtttctggttttaacgcaagaatccctcacatcccaaaaatcgtcgagctagatcatttgaccatcactggtaacgtctttttaggtaaagatgtcactttgaggggtactgtcatcatcgtttgctccgacggtcataaaatcgatattccaaacggctccatattggaaaatgttgtcgttactggtaatttgcaaatcttggaacattga

SEQ ID NO: 57 - protein, 499 aa, Saccharomyces cerevisiae
  Amino acid sequence of UTP--glucose-1-phosphate uridylyltransferase (UGP1) originating from Saccharomyces cerevisiae
  Amino acid sequence of UTP--glucose-1-phosphate uridylyltransferase (UGP1) originating from Saccharomyces cerevisiae
MSTKKHTKTHSTYAFESNTNSVAASQMRNALNKLADSSKLDDAARAKFENELDSFFTLFRRYLVEKSSRTTLEWDKIKSPNPDEVVKYEIISQQPENVSNLSKLAVLKLNGGLGTSMGCVGPKSVIEVREGNTFLDLSVRQIEYLNRQYDSDVPLLLMNSFNTDKDTEHLIKKYSANRIRIRSFNQSRFPRVYKDSLLPVPTEYDSPLDAWYPPGHGDLFESLHVSGELDALIAQGREILFVSNGDNLGATVDLKILNHMIETGAEYIMELTDKTRADVKGGTLISYDGQVRLLEVAQVPKEHIDEFKNIRKFTNFNTNNLWINLKAVKRLIESSNLEMEIIPNQKTITRDGHEINVLQLETACGAAIRHFDGAHGVVVPRSRFLPVKTCSDLLLVKSDLFRLEHGSLKLDPSRFGPNPLIKLGSHFKKVSGFNARIPHIPKIVELDHLTITGNVFLGKDVTLRGTVIIVCSDGHKIDIPNGSILENVVVTGNLQILEH

SEQ ID NO: 58 - DNA, 480 bp, Saccharomyces cerevisiae
  "Nucleic acid sequence of Glucosamine 6-phosphate N-acetyltransferase (GNA1) originating from Saccharomyces cerevisiae"
  Nucleic acid sequence of Glucosamine 6-phosphate N-acetyltransferase (GNA1) originating from Saccharomyces cerevisiae
atgagcttacccgatggattttatataaggcgaatggaagagggggatttggaacaggtcactgagacgctaaaggttttgaccaccgtgggcactattacccccgaatccttcagcaaactcataaaatactggaatgaagccacagtatggaatgataacgaagataaaaaaataatgcaatataaccccatggtgattgtggacaagcgcaccgagacggttgccgctacggggaatatcatcatcgaaagaaagatcattcatgaactggggctatgtggccacatcgaggacattgcagtaaactccaagtatcagggccaaggtttgggcaagctcttgattgatcaattggtaactatcggctttgactacggttgttataagattattttagattgcgatgagaaaaatgtcaaattctatgaaaaatgtgggtttagcaacgcaggcgtggaaatgcaaattagaaaatag

SEQ ID NO: 59 - protein, 159 aa, Saccharomyces cerevisiae
  Amino acid sequence of Glucosamine 6-phosphate N-acetyltransferase (GNA1) originating from Saccharomyces cerevisiae
  Amino acid sequence of Glucosamine 6-phosphate N-acetyltransferase (GNA1) originating from Saccharomyces cerevisiae
MSLPDGFYIRRMEEGDLEQVTETLKVLTTVGTITPESFSKLIKYWNEATVWNDNEDKKIMQYNPMVIVDKRTETVAATGNIIIERKIIHELGLCGHIEDIAVNSKYQGQGLGKLLIDQLVTIGFDYGCYKIILDCDEKNVKFYEKCGFSNAGVEMQIRK

SEQ ID NO: 60 - DNA, 1674 bp, Saccharomyces cerevisiae
  "Nucleic acid sequence of phosphoacetylglucosamine mutase (PCM1) originating from Saccharomyces cerevisiae"
  Nucleic acid sequence of phosphoacetylglucosamine mutase (PCM1) originating from Saccharomyces cerevisiae
atgaaggttgattacgagcaattgtgcaaactctacgatgacacgtgccgcacaaagaatgtgcagttcagttacggtacggccggattcagaacgctggccaagaatttggatacggtgatgttcagtactggtatactggcggttctcaggtcgctgaagcttcagggtcagtatgtgggggtgatgatcacggcgtcgcacaacccataccaggacaacggggtcaagatcgtggaaccagacggatcgatgcttttggccacatgggagccatatgccatgcagttggccaatgcggcctcttttgccactaattttgaagaatttcgtgttgagttggccaagctgattgaacacgaaaagattgatttgaatacaaccgtcgtgcctcacatcgtggttgggagagactctagggaaagtagtccatacttgctgcgctgcttgacttcctccatggccagcgtcttccacgcgcaagttttggacctaggctgtgtcactacgcctcaattgcattacattactgatttgtccaacaggcggaaactggaaggagacacagcgccagttgccacagaacaggactactattcgttctttataggagccttcaacgagctcttcgccacgtatcagctggagaagaggctgtctgtcccaaaattgttcatagacacagccaatggtatcggtggtccacagttgaaaaaactactggcctccgaagattgggacgtgccagcggagcaagttgaggtaatcaacgacaggtccgatgttccagaactgttgaattttgaatgcggtgcggattatgtgaagactaaccagagattacccaagggtctttctccatcctcgtttgattcgctatattgctcctttgatggtgacgcagacagggttgtgttctactatgtcgactcaggatcaaaatttcatttgttggatggtgacaaaatttccactttgtttgcaaagttcttgtctaaacaactagaattggcacacctagaacattctttgaagattggtgttgtgcaaactgcctatgcaaacggcagttccaccgcttacataaaaaatacgttgcactgtcccgtgtcttgcactaagacaggtgttaaacacttgcatcatgaagctgccactcagtacgatattggcatttatttcgaagcaaatggacatggtacgattatattcagcgaaaaatttcatcgaactatcaaatctgaattatccaagtccaagttaaatggtgatacgttagctttgagaactttgaagtgtttctctgaattgattaatcagaccgtgggagatgctatttcagacatgcttgctgtccttgctactttggcgattttgaaaatgtcgccaatggattgggatgaagagtatactgatttgcccaacaagctggttaagtgcatcgttcctgataggtcaattttccaaaccacggaccaggaaagaaaattgctcaatccagtggggttgcaagacaagatagatcttgtggtagccaagtatcccatgggaagaagctttgtcagagccagtggtacggaggatgcggtgagggtttatgcggaatgtaaggactcctctaagttaggtcaattttgtgacgaagtggtggagcacgttaaggcatctgcttga

SEQ ID NO: 61 - protein, 557 aa, Saccharomyces cerevisiae
  Amino acid sequence of phosphoacetylglucosamine mutase (PCM1) originating from Saccharomyces cerevisiae
  Amino acid sequence of phosphoacetylglucosamine mutase (PCM1) originating from Saccharomyces cerevisiae
MKVDYEQLCKLYDDTCRTKNVQFSYGTAGFRTLAKNLDTVMFSTGILAVLRSLKLQGQYVGVMITASHNPYQDNGVKIVEPDGSMLLATWEPYAMQLANAASFATNFEEFRVELAKLIEHEKIDLNTTVVPHIVVGRDSRESSPYLLRCLTSSMASVFHAQVLDLGCVTTPQLHYITDLSNRRKLEGDTAPVATEQDYYSFFIGAFNELFATYQLEKRLSVPKLFIDTANGIGGPQLKKLLASEDWDVPAEQVEVINDRSDVPELLNFECGADYVKTNQRLPKGLSPSSFDSLYCSFDGDADRVVFYYVDSGSKFHLLDGDKISTLFAKFLSKQLELAHLEHSLKIGVVQTAYANGSSTAYIKNTLHCPVSCTKTGVKHLHHEAATQYDIGIYFEANGHGTIIFSEKFHRTIKSELSKSKLNGDTLALRTLKCFSELINQTVGDAISDMLAVLATLAILKMSPMDWDEEYTDLPNKLVKCIVPDRSIFQTTDQERKLLNPVGLQDKIDLVVAKYPMGRSFVRASGTEDAVRVYAECKDSSKLGQFCDEVVEHVKASA

SEQ ID NO: 62 - DNA, 574 bp, Artificial Sequence
  "Nucleic acid sequence of promotor pTDH3"
  Nucleic acid sequence of promotor pTDH3
ctgctgtaacccgtacatgcccaaaatagggggcgggttacacagaatatataacatcgtaggtgtctgggtgaacagtttattcctggcatccactaaatataatggagcccgctttttaagctggcatccagaaaaaaaaagaatcccagcaccaaaatattgttttcttcaccaaccatcagttcataggtccattctcttagcgcaactacagagaacaggggcacaaacaggcaaaaaacgggcacaacctcaatggagtgatgcaacctgcctggagtaaatgatgacacaaggcaattgacccacgcatgtatctatctcattttcttacaccttctattaccttctgctctctctgatttggaaaaagctgaaaaaaaaggttgaaaccagttccctgaaattattcccctacttgactaataagtatataaagacggtaggtattgattgtaattctgtaaatctatttcttaaacttcttaaattctacttttatagttagtcttttttttagttttaaaacaccaagaacttagtttcgaataaacacacataaacaaacaaa

SEQ ID NO: 63 - DNA, 585 bp, Saccharomyces kudriavzevii
  "Nucleic acid sequence of promotor pTDH3.Sk"
  Nucleic acid sequence of promotor pTDH3.Sk
caattcatcggcccttttagcggctacccgcgccatctaaatgatagggcgggtgacactatggtaaatcccataattaggtgtctgggtgagtggttctgatgccggcatccactaaatatattggagcccattttttacgcgggcttccagaaaaaaagagaatcccagcaccaaaaggtggttctcttcaccaaccatcagatcataggtccacaaccacacataacaggggcacaaaaaggcaaaaaacggacataacctcaatggagtgatgcaaattgactggagcaaaagctgacacaaggcattgattgacctacgcatgtatctgtattcttttcttacaccttctattaccttctaactctttgggttggaaaaaactgaaaaaaaaggttgggacctggttcccccaagttgtccccctacttggttattaaatatataaagacagcaagtgttgattataatcttgtaaatctatagttcttaatctatacttctatttatattttaaattagtctttttatttccaagtccccaagaacttagtttcgaataaacacacacaaataaacaca

SEQ ID NO: 64 - DNA, 700 bp, Saccharomyces bayanus
  "Nucleic acid sequence of promotor pTDH3-1.sba"
  Nucleic acid sequence of promotor pTDH3-1.sba
gcagcgcttcttccgctctagtttttatagttattattactaccaccttaaaaatacgtaaatactcaaaatagtagtgatattcccaaccttattcatccaaggcacatcatcatcatcagccattcatctttcacctgccattagtaacccgtcttctcattgagcgggttacggcagccacaggccacattccgaatgtctgggtgagcggtcccttttccagcatccactaaatatctccgatcccgctttttaatctggcttcctgaaaaaaagagaatcccagcaccaaaaaatggctctcttcaccaaccatcagatcataggtcccattctcttaccgcaaccgtacagaacaggggaaaacgggtacaacctcaatggagtgatgcaaactgactggagcaaaaagctgacacaaggcaatcgacctacgtgtctgtctattttctcacaccttctattaccttctaactctctgggttggaaaaaactgaaaaaaaggttgagaccagtttccacaaatcatccccctgtttgattaataaatatataaagacgacaactatcgatcataaactcataaaactataactcctttacacttcttattttatagttattctattttaattcttattgattttaaaaccccaagaacttagtttcgaaaacacacacacacaaacaattaaaa

SEQ ID NO: 65 - DNA, 602 bp, Saccharomyces arboricola
  "Nucleic acid sequence of promotor pTDH3.Sar"
  Nucleic acid sequence of promotor pTDH3.Sar
gagctaaatatcagcccttcgggtcctgcctgctacccggtcctgttcgaataaaaacgcgggtaacacgacccagtaacacctgtcgttgggtgtctgggtcagaagttctgataccggcttccactaaatagattgggttccgctctttacgctggcttcctgaaaaaagagattccgggcaccaaaaaattggtctctttgccaaccatcagatcataggtccattctcttaccataaccacacaggataggggcaccacaggcgaaaatgggcacaaaatctcaatggagtgatgcaaattagctggaacaaaagctgacacaaggcaattaacctgcgcatgtatccatctccttttcttacaccttctcttacgttctaactgtttgggttggaaaaattaaaaaaaaaaggttgagaccagtttccccaaatcgtccccctacttgattcataaatatataaagacgacaactattgattataatcttgtaaatctataactctttactttctcctatttataatttaacttaatctttttagatttaaaaccccaagaacttagtttcgaacaaacacacacaaataaacaaaa

SEQ ID NO: 66 - DNA, 550 bp, Artificial Sequence
  "Nucleic acid sequence of promotor pENO2"
  Nucleic acid sequence of promotor pENO2
cgctcagcatctgcttcttcccaaagatgaacgcggcgttatgtcactaacgacgtgcaccaacttgcggaaagtggaatcccgttccaaaactggcatccactaattgatacatctacacaccgcacgccttttttctgaagcccactttcgtggactttgccatatgcaaaattcatgaagtgtgataccaagtcagcatacacctcactagggtagtttctttggttgtattgatcatttggttcatcgtggttcattaattttttttctccattgctttctggctttgatcttactatcatttggatttttgtcgaaggttgtagaattgtatgtgacaagtggcaccaagcatatataaaaaaaaaaagcattatcttcctaccagagttgattgttaaaaacgtatttatagcaaacgcaattgtaattaattcttattttgtatcttttcttcccttgtctcaatcttttatttttattttatttttcttttcttagtttctttcataacaccaagcaactaatactataacatacaataata

SEQ ID NO: 67 - DNA, 598 bp, Artificial Sequence
  "Nucleic acid sequence of promotor pTEF3"
  Nucleic acid sequence of promotor pTEF3
ggctgataatagcgtataaacaatgcatactttgtacgttcaaaatacaatgcagtagatatatttatgcatattacatataatacatatcacataggaagcaacaggcgcgttggacttttaattttcgaggaccgcgaatccttacatcacacccaatcccccacaagtgatcccccacacaccatagcttcaaaatgtttctactccttttttactcttccagattttctcggactccgcgcatcgccgtaccacttcaaaacacccaagcacagcatactaaatttcccctctttcttcctctagggtgtcgttaattacccgtactaaaggtttggaaaagaaaaaagagaccgcctcgtttctttttcttcgtcgaaaaaggcaataaaaatttttatcacgtttctttttcttgaaaatttttttttttgatttttttctctttcgatgacctcccattgatatttaagttaataaacggtcttcaatttctcaagtttcagtttcatttttcttgttctattacaactttttttacttcttgctcattagaaagaaagcatagcaatctaatctaagttttaattacaaa

SEQ ID NO: 68 - DNA, 383 bp, Artificial Sequence
  "Nucleic acid sequence of promotor pTEF1"
  Nucleic acid sequence of promotor pTEF1
gtttagcttgcctcgtccccgccgggtcacccggccagcgacatggaggcccagaataccctccttgacagtcttgacgtgcgcagctcaggggcatgatgtgactgtcgcccgtacatttagcccatacatccccatgtataatcatttgcatccatacattttgatggccgcacggcgcgaagcaaaaattacggctcctcgctgcagacctgcgagcagggaaacgctcccctcacagacgcgttgaattgtccccacgccgcgcccctgtagagaaatataaaaggttaggatttgccactgaggttcttctttcatatacttccttttaaaatcttgctacgatacagttctcacatcacatccgaacataaacaacc

SEQ ID NO: 69 - DNA, 383 bp, Ashbya gossypii; identical to SEQ ID NO: 68
  "Nucleic acid sequence of promotor pTEF1.ago"
  Nucleic acid sequence of promotor pTEF1.ago

SEQ ID NO: 70 - DNA, 498 bp, Saccharomyces bayanus
  "Nucleic acid sequence of promotor pTEF1.Sba"
  Nucleic acid sequence of promotor pTEF1.Sba
cgccaacaaaccttcgaacactttaattttcgaggaccgcagatcctcacatcacacccacacccaagactgcttcccccacacaccctgcatctgtacactttcttctgctctgtttttctctccggcgttctctcgggtcgcccgcatcgccgcgccggctggaaccgcccacgcaccgcatattgcaaatcgcctgccccctcttgctcctttttgagggcgcgccgttacccgcgcccagggtccggaaaaagaaacaaggctctaccgcgtttctttttccttgtcgaaaaaggcaaaaatgaaaatttttatcacgtttctttttttttgaaaaattttttttttggttttttttctttcgatggcctcccattgatatttaagttaataaatggttttcagttttcaagtttcagtttgtgttcttctttgctaactttcacttacacctcgaaagaaagtatagcaatctaatcttagttttaattacaa

SEQ ID NO: 71 - DNA, 76 bp, Artificial Sequence
  "Nucleic acid sequence of promotor pPDC1"
  Nucleic acid sequence of promotor pPDC1
ttatttacctatctctaaacttcaacaccttatatcataactaatatttcttgagataagcacactgcacccatac

SEQ ID NO: 72 - DNA, 998 bp, Artificial Sequence
  "Nucleic acid sequence of promotor pCCW12"
  Nucleic acid sequence of promotor pCCW12
aaccagggcaaagcaaaataaaagaaacttaatacgttatgccgtaatgaagggctaccaaaaacgataatctcaactgtaaacaggtacaatgcggacccttttgccacaaaacatacatcattcattgccggaaaaagaaagaagtgaagacagcagtgcagccagccatgttgcgccaatctaattatagatgctggtgccctgaggatgtatctggagccagccatggcatcatgcgctaccgccggatgtaaaatccgacacgcaaaagaaaaccttcgaggttgcgcacttcgcccacccatgaaccacacggttagtccaaaaggggcagttcagattccagatgcgggaattagcttgctgccaccctcacctcactaacgctgcggtgtgcggatacttcatgctatttatagacgcgcgtgtcggaatcagcacgcgcaagaaccaaatgggaaaatcggaatgggtccagaactgctttgagtgctggctattggcgtctgatttccgttttgggaatcctttgccgcgcgcccctctcaaaactccgcacaagtcccagaaagcgggaaagaaataaaacgccaccaaaaaaaaaaataaaagccaatcctcgaagcgtgggtggtaggccctggattatcccgtacaagtatttctcaggagtaaaaaaaccgtttgttttggaattccccatttcgcggccacctacgccgctatctttgcaacaactatctgcgataactcagcaaattttgcatattcgtgttgcagtattgcgataatgggagtcttacttccaacataacggcagaaagaaatgtgagaaaattttgcatcctttgcctccgttcaagtatataaagtcggcatgcttgataatctttctttccatcctacattgttctaattattcttattctcctttattctttcctaacataccaagaaattaatcttctgtcattcgcttaaacactatatcaata

SEQ ID NO: 73 - DNA, 976 bp, Saccharomyces mikatae
  "Nucleic acid sequence of promotor pCCW12.Sm"
  Nucleic acid sequence of promotor pCCW12.Sm
cgttgtgctgtagtgaaggaagactaaaaaggataatcacagttgtaaagaggtataatgcggacccttttgccacaaaacacacatctttcgtttccaaaataagaaagaagaaagcaaaaagattagcagccacgttgctgcgatctaattatagacggtggcgtcatcattctcacccaagattgtgtcttgaacctgccacgggtcctgcgttatcgccggatgtaaaactagacatgcaaaaaaaggaccttccaggtagcgtgctccacaccacccatgaccaccacagttagtccaaaagaggcagcaccacttcccgatgggggaattagattgctgccaccctcacctcactaatgctgcggtgtgcggatatgccctgctatatatagctccgcgtttttgaaccagcacagcgcgagcaccaaaaaggaaaatcgcataggcccagaactgatttcagcacgggctattggcgttgggtttccgttctgggaaaccttcgccgcgtccccctcacaaacctccgcacaagttcgagcaagcgggaaaaaacgaaaaacgccattaatactaaataaagcaaatcctcgaagcgtgggtggcaagcccctggatttttccgcacaagtactcttctcaggagtaaaaaaacccgtttgttttggaattccccatttcgcggccatctacgccggtatcttcgcaatatctatcagcgataactcagcaattttaatattcgtgttgcagtgctgcgatagcgggagtcttgtttgtaacataacggcagaaaggaatgagagaaaattttccattctttggcctccgttcaagtatataaagccggcatgcttggtaatctttctctctcttctgtattgtttctataatacttttatcttctaattattttctgaaaaaaccaagaaattaatcttctgtcattcgcttaaacactatatcaata

SEQ ID NO: 74 - DNA, 750 bp, Saccharomyces kudriavzevii
  "Nucleic acid sequence of promotor pCCW12.Sk"
  Nucleic acid sequence of promotor pCCW12.Sk
tgtaaaatcctacacgcaaaaaacctcttgggttgcgcgttttccaccacccacgacccgcacaatcaatccaaaaggggcaacgccagttcccaatgcgggaattagctcctcacccccctcacccgctaacgctgcggtgtgcggacacgcagcagtatttatagatcctcgtgttggaaccagcccgcgtgagcaccaaattggaaagtcgcaatgggcccagaaccgctttcagtactgggccattggcgtctagtttccgttttgagcgtccttcgccgcgtctctctgtgaaatccccgcacaagtctgagcaggcaaaaaaaaaaaacgccaccaaaaataaataaagccaatcctcgaaggatgagtaggaaaggaagcccctggttttttcccgcacgaatatttttcaggagtgaaaaaatccgtttgttttggaattccccatttcgcgctcacctacgccggtatctttggaacaactatcagcgataactcagcaaaatttgcatatccgtgctgcaatagtgcgatagtgggattgggagtcttgttgcatcataacggcagaaaggaatgaataaaaattttccgttctttgtctccgttcaagtatataaagtcggcatgcttgattatcttttcttctcttctactacatttctatttcactttctactctattcttccctgaaaaacccaagaaaataatcttctgtcattcgcttaaacaatatatcaaaa

SEQ ID NO: 75 - DNA, 750 bp, Saccharomyces bayanus
  "Nucleic acid sequence of promotor pCCW12.Sba"
  Nucleic acid sequence of promotor pCCW12.Sba
accatgccacggtgctggccccacttccacccacgacccgcacggttggcccgaaaggggcaacaccagttcccaatacggaaattagtccgccaccaccctcacctcgctagagctgcggtgtgcgggcgtgcatcgctatttatagacatgcctgctggcgtcaccgcgcgcgagcaccaaacaggaaaatcgcactgggcccagaaccacgctatgcgctgggccgatggcgtccggtttccctttgggagccccctgccacgttcgcctaacaaatccccgcaccggcttgagaaaaaagcgaaaagcgaaaaaaaaaaatcaacgccaccaaaattaaaaaaaaagagccatcctcgaagggtgaatagtagcccctgacttttcccgcacagacagacacctttcaggagtgaacaaaaaagcagtttgttttggaattcccccatttcgcggtggcctgcgcaggtatctctgcgtcaactatcagcgataactcagcaaattttgcatattcgtgttgcgatactacgataatgggagtctgtcgcctaataacggcaacaaggaatgagagagaaaaattttcttcattctccagctcccgttcaagtatataaggtcggcatggtcgattgtctttccttctcttcagttacgtctctctatttacattattcttatttttatttaataaaaaccccaagaaattaatcttctgtcattcgcttaaacactatatcaaaa

SEQ ID NO: 76 - DNA, 750 bp, Saccharomyces arboricola
  "Nucleic acid sequence of promotor pCCW12.Sar"
  Nucleic acid sequence of promotor pCCW12.Sar
aaaaaacaaccttctgccaacctgcgtgcttctcaccacccatgacccacacaattgacccgaatggggcaactccagttcccaatacgggaattaactcgccaccatatttaccgcgttgaagctgtggtgtgcggacactccgtactatttatagacccacgcggtggaaccagcacgcgcgcgcactaaacaggaaaatcgcattgagtccagaaccgccaccagcacttggccattggcgtctaatttccgttttcggcgcccctcaccgcgtccttctaacaaagcgcgcacaagcttgagcaagtgaaaagaaaattaaaaataaaaaaccgccaccaaaacaaataaagcaatcttcgaagtgtgggttggtgggaagcccctggcttttcccgcaccagtcgttttcaggagtaaaaaaatacccgtttgttttggaattccccatttcgcggcgacctgcgccggtatctttgcaacaactatttgcgataactcagcaaaatttgcatattcgtgttgggatattgcgatagtgggagtcttgttgcataataacggtaaaaagaagtgaaggaaaaaaatttgcatcctttagtctcagttcaagtatataaagtcgggatattcaattatctttctttctcttgctcaaaggtttctatattttttttatagtatttcttttgttataaaataccaagaaattaatcttctgtcattcgcttaaatactacatcaata

SEQ ID NO: 77 - DNA, 500 bp, Artificial Sequence
  "Nucleic acid sequence of promotor pNUP57"
  Nucleic acid sequence of promotor pNUP57
tcatctgcgcaatgactatcaagaccttctgcaagaatttcaaatctcactgaaaatcttgaccgaaaagtgtcttgaaaacccatcaagcctgcaaaacctatctttgacattagtctccattataaaaacggcatagttgggagaaaactttccatacttcaattgtggactgatataagtattttagttttgcccgcatgatcatcccacatggctacagcagttctctcataggaaaatagtacaatagctacgtgatataatctaaataattgttgccaatgtgtaattatatcattttgaacgtacgcgaaatggattattttcaaaaattttgtttcttgaaatgagtaaaagcaaaagtccaactctccaagtcgatgtaaacaactttttgccaaagggactgaaagactaaatcgaggattatcccgttcaaactattccagaaacgctcgttagtaacaaaagacataccttgttgaccaattgatcac

SEQ ID NO: 78 - DNA, 523 bp, Ashbya gossypii
  "Nucleic acid sequence of promotor pCCW10.ago"
  Nucleic acid sequence of promotor pCCW10.ago
ggtaccacggcaacctcgttcgctgttcatccccttcgtcacacaggacgttggatgccgtaagcagcgttgcttttgatcctcaggatcggccgggtaacccgcggctgcttctattttagtattcatatctcaagcacatccattccggccgtttgggggcgccgccgcactcgtgtccattcctaccgtggcacttagggctatcctgtcggagcgccccgccgaccgccttatcggcaccaaaagtagaagccccggccccgcgtggctcagactcaccatcggtgctatttacttttcgatcagatcgcggcgcgcggtggccggcatttccggaagcggccacggagcagaggtggcgcattcgaatcgcatacgtcttcgccacgccggaaaaaaaattttcggctatataaggagaggcggccgtcttgctgcaggcagtttcactttctctaaaaccaaagaacatcgatttctttagtcactcgcttccttacaccgaactcgaggcggccgc

SEQ ID NO: 79 - DNA, 943 bp, Artificial Sequence
  "Nucleic acid sequence of promotor pCWP2"
  Nucleic acid sequence of promotor pCWP2
ctagcctcccctttttattttgtgcggtcaccgcaagggacaaagcttttcttagaaaaccgtctgagaagcataacgtacgccatcccctagacatattaataatgctacagatactatgctgctcgtctttttttgacgacccttttattgcaatgtgcaactaatggcaaacaaccacatagtatcacagtattacattgcctccaccgatgcggatgttagggcgccaagtctgtcatgaagcatgttcctgtcataatcttgtatgcaaaataccgcgttctgcgccactgatatgctaggcagcagcaacctatgcagaagattgcttttcccacgcctgttttacgtctccagggcacttgaaacaatgcagcgatcgccgccacaacacgccaaagagaagcgaaagtgggcctgggcggcctcagtttcggcagaggtaaacaacacgaactgaactgccttagctccgaagggcaattccacaggcactccgcggggcccggccaaggcccaaaaggcgtggaatatgcgcgttttggggccataacacccagtaccacggccggaacgggccatataataagtttttcactctcaagaatggtaaacgtaaataggaacatcccactaccctagaaattgcggaaatttcgcgcttatcattagaaaatctggaaccgtcctttttcctctttcttgcatttccctttccgtattattgccattctttaactgcatttggggaaccgtagaccaaaagccaaacagagaaatgtaacgttctaaaaaaaaaacaacgaaaaaattgaaaaataagatacaataatcgtatataaatcaggcttcttgttcatcattttcaattctcttcttgccatcccttttcctatctttgttcttttcttctcataatcaagaataaataacttcatca

SEQ ID NO: 80 - DNA, 535 bp, Artificial Sequence
  "Nucleic acid sequence of promotor pRPLA1"
  Nucleic acid sequence of promotor pRPLA1
tcaagttggatactgatctgatctctccgccctactaccagggaccctcatgattaccgctcgaatgcgacgtttcctgcctcataaaactggcttgaaaatatttattcgctgaacagtagcctagcttataaaaatttcatttaattaatgtaatatgaaaactcacatgccttctgtttctaaaattgtcacagcaagaaataacattaccatacgtgatcttattaaactctagtatcttgtctaatacttcatttaaaagaagccttaaccctgtagcctcatctatgtctgctacatatcgtgaggtacgaatatcgtaagatgataccacgcaactttgtaatgattttttttttttcattttttaaagaatgcctttacatggtatttgaaaaaaatatctttataaagtttgcgatctcttctgttctgaataatttttagtaaaagaaatcaaaagaataaagaaatagtccgctttgtccaatacaacagcttaaaccgattatctctaaaataacaagaagaa

SEQ ID NO: 81 - DNA, 505 bp, Artificial Sequence
  "Nucleic acid sequence of promotor pCUP1"
  Nucleic acid sequence of promotor pCUP1
cggcaaacttcaacgatttctatgatgcattttataattagtaagccgatcccattaccgacatttgggcgctatacgtgcatatgttcatgtatgtatctgtatttaaaacacttttgtattatttttcctcatatatgtgtataggtttatacggatgatttaattattacttcaccaccctttatttcaggctgatatcttagccttgttactagttagaaaaagacatttttgctgtcagtcactgtcaagagattcttttgctggcatttcttctagaagcaaaaagagcgatgcgtcttttccgctgaaccgttccagcaaaaaagactaccaacgcaatatggattgtcagaatcatataaaagagaagcaaataactccttgtcttgtatcaattgcattataatatcttcttgttagtgcaatatcatatagaagtcatcgaaatagatattaagaaaaacaaactgtacaatcaatcaatcaatcatcacataaa

SEQ ID NO: 82 - DNA, 510 bp, Artificial Sequence
  "Nucleic acid sequence of promotor pMET6"
  Nucleic acid sequence of promotor pMET6
ccacaggaaatatttcacgtgacttacaaacagagtcgtacgtcaggaccggagtcaggtgaaaaaatgtgggccggtaaagggaaaaaaccagaaacgggactactatcgaactcgtttagtcgcgaacgtgcaaaaggccaatatttttcgctagagtcatcgcagtcatggcagctctttcgctctatctcccggtcgcaaaactgtggtagtcatagctcgttctgctcaattgagaactgtgaatgtgaatatggaacaaatgcgatagatgcactaatttaagggaagctagctagttttcccaactgcgaaagaaaaaaaggaaagaaaaaaaaattctatataagtgatagatatttccatctttactagcattagtttctcttttacgtattcaatatttttgttaaactcttcctttatcataaaaaagcaagcatctaagagcattgacaacactctaagaaacaaaataccaatataatttcaaagtacatatcaaaa

SEQ ID NO: 83 - DNA, 686 bp, Artificial Sequence
  "Nucleic acid sequence of promotor pMET25"
  Nucleic acid sequence of promotor pMET25
ttacattatcaatccttgcgtttcagcttccactaatttagatgactatttctcatcatttgcgtcatcttctaacaccgtatatgataatatactagtaacgtaaatactagttagtagatgatagttgatttttattccaacactaagaaataatttcgccatttcttgaatgtatttaaagatatttaatgctataatagacatttaaatccaattcttccaacatacaatgggagtttggccgagtggtttaaggcgtcagatttaggtggatttaacctctaaaatctctgatatcttcggatgcaagggttcgaatcccttagctctcattattttttgctttttctcttgaggtcacatgatcgcaaaatggcaaatggcacgtgaagctgtcgatattggggaactgtggtggttggcaaatgactaattaagttagtcaaggcgccatcctcatgaaaactgtgtaacataataaccgaagtgtcgaaaaggtggcaccttgtccaattgaacacgctcgatgaaaaaaataagatatatataaggttaagtaaagcgtctgttagaaaggaagtttttcctttttcttgctctcttgtcttttcatctactatttccttcgtgtaatacagggtcgtcagatacatagatacaattctattacccccatccataca

SEQ ID NO: 84 - DNA, 363 bp, Artificial Sequence
  "Nucleic acid sequence of promotor pSAM1"
  Nucleic acid sequence of promotor pSAM1
gaaacggacgtaagacggaaatagaatttgaagataaagttatatatcactacacacgaatactttcttttttttttttcacaggaaaactgtggtggcgcccttgcctactagtgcatttcttttttcgggttcttgtctcgacgaaattttagcctcatcgtagtttttcactctggtatcgatgaaaaagggaagagtaaaaagttttccgtttagtacttaatgggattggtttgggacgtatatatcgactggtgttgtctgttattcatcgttgtttttcggttagcttcgaaaaaaaaatagagtaaaaaccaggaatttaccctaaaaacaagaaaaaataagataaacgaaaat

SEQ ID NO: 85 - DNA, 300 bp, Artificial Sequence
  "Nucleic acid sequence of terminator tTPI1"
  Nucleic acid sequence of terminator tTPI1
gattaatataattatataaaaatattatcttcttttctttatatctagtgttatgtaaaataaattgatgactacggaaagcttttttatattgtttctttttcattctgagccacttaaatttcgtgaatgttcttgtaagggacggtagatttacaagtgatacaacaaaaagcaaggcgctttttctaataaaaagaagaaaagcatttaacaattgaacacctctatatcaacgaagaatattactttgtctctaaatccttgtaaaatgtgtacgatctctatatgggttactca

SEQ ID NO: 86 - DNA, 299 bp, Artificial Sequence
  "Nucleic acid sequence of terminator tMET25"
  Nucleic acid sequence of terminator tMET25
gtgtgcgtaatgagttgtaaaattatgtataaacctactttctctcacaagtactatacttttataaaacgaactttattgaaatgaatatcctttttttcccttgttacatgtcgtgactcgtactttgaacctaaattgttctaacatcaaagaacagtgttaattcgcagtcgagaagaaaaatatggtgaacaagactcatctacttcatgagactactttacgcctcctataaagctgtcacactggataaatttattgtaggaccaagttacaaaagaggatgatggaggttt

SEQ ID NO: 87 - DNA, 300 bp, Artificial Sequence
  "Nucleic acid sequence of terminator tDIT1"
  Nucleic acid sequence of terminator tDIT1
taaagtaagagcgctacattggtctacctttttgttcttttacttaaacattagttagttcgttttctttttctcatttttttatgtttcccccccaaagttctgattttataatattttatttcacacaattccatttaacagagggggaatagattctttagcttagaaaattagtgatcaatatatatttgcctttcttttcatcttttcagtgatattaatggtttcgagacactgcaatggccctagttgtctaagaggatagatgttactgtcaaagatgatattttgaatttc

SEQ ID NO: 88 - DNA, 300 bp, Artificial Sequence
  "Nucleic acid sequence of terminator tRPL3"
  Nucleic acid sequence of terminator tRPL3
gaagttttgttagaaaataaatcattttttaattgagcattcttattcctattttatttaaatagttttatgtattgttagctacatacaacagtttaaatcaaattttctttttcccaagtccaaaatggaggtttattttgatgacccgcatgcgattatgttttgaaagtataagactacatacatgtacatatatttaaacatgtaaacccgtccattatattgcttactttcttcttttttgccgttttgacttggacctctggtttgctatttccttacaatctttgctacaat

SEQ ID NO: 89 - DNA, 304 bp, Saccharomyces mikatae
  "Nucleic acid sequence of terminator tRPL3.sm"
  Nucleic acid sequence of terminator tRPL3.sm
gaagtttttaaagcattttttagacacttctcatttttctaagtttttttaaaatagttttatgtatttactacgtatcacaatttgaaataattcatcttcccaaaaaactaagatttttatccttgtcacgatccgtaaccagtttataatattttagagcttatacacgtacgtatacacacgtgtcggtacatgagaattacgttcaaaattattcactttttttttctctgccgttttacttttgaactctgtctcgctatttccttacaatcttcgctacaataccacttgcccttgg

SEQ ID NO: 90 - DNA, 299 bp, Saccharomyces bayanus
  "Nucleic acid sequence of terminator tRPL3.sba"
  Nucleic acid sequence of terminator tRPL3.sba
gaagttttctgacaaaaacataacgttttttccaatcatttcttatttttccggtttatttaaatagtttttatgtactattatacgtatgactatttaacttaaattcttcctcccaagaaatctcccaagtttttcattatcatggcatacaccactatcagttacaaaatggtagctcaaccatatatatatctctatatacacatataaatgcaaacaggtccaagtcaccgctcactgcagtttcttttgccgttttgacttcgatctctgcttggctattttctcacaatcct

SEQ ID NO: 91 - DNA, 300 bp, Artificial Sequence
  "Nucleic acid sequence of terminator tRPL41B"
  Nucleic acid sequence of terminator tRPL41B
gcggattgagagcaaatcgttaagttcaggtcaagtaaaaattgatttcgaaaactaatttctcttatacaatcctttgattggaccgtcatcctttcgaatataagattttgttaagaatattttagacagagatctactttatatttaatatctagatattacataatttcctctctaataaaatatcattaataaaataaaaatgaagcgatttgattttgtgttgtcaacttagtttgccgctatgcctcttgggtaatgctattattgaatcgaagggctttattatattaccct

SEQ ID NO: 92 - DNA, 300 bp, Artificial Sequence
  "Nucleic acid sequence of terminator tRPL15A"
  Nucleic acid sequence of terminator tRPL15A
gctggttgatggaaaatataattttattgggcaaacttttgtttatctgatgtgttttatactattatctttttaattaatgattctatatacaaacctgtatattttttctttaaccaatttttttttttatagacctagagctgtacttttattctgctatcaagcaaacccctaccccctcttctcaatcctcccctcaggcagaacttatctacctgtatcaaggagcggacgagggagtcctaattgttctacgtataccaatgctagcagcttacataggtggtggcactacca

SEQ ID NO: 93 - DNA, 300 bp, Saccharomyces bayanus
  "Nucleic acid sequence of terminator tRPL15A.sba"
  Nucleic acid sequence of terminator tRPL15A.sba
gctggctgatgaaaaatatagttctgttgggcaagcatttgtttacctagcatctcttttatactattattatctttatatttgatgattttatatacaagttgtataccttttctttaaccaatttttttttttctaatggtgcacctagaagtacattttttctcaccaatagatagtcaagatactcccagcctctatggcgttaccacggagccgacaagggaaagctgcttatcttacatatgcagatgccaaggcccgttacaggccgccttattgatgtttagaaatagcttc

SEQ ID NO: 94 - DNA, 300 bp, Artificial Sequence
  "Nucleic acid sequence of terminator tIDP1"
  Nucleic acid sequence of terminator tIDP1
tcgaatttacgtagcccaatctaccacttttttttttcattttttaaagtgttatacttagttatgctctaggataatgaactacttttttttttttttttttactgttatcataaatatatataccttattgttgtttgcaaccgtcggttaattccttatcaaggttccccaagttcggatcattaccatcaatttccaacattttcatgagttcttcttcttcattaccgtgttttagggggctgttcgcacttctaatagggctatcaccaagctgttctaattcgtccaaaagtt

SEQ ID NO: 95 - DNA, 300 bp, Saccharomyces bayanus
  "Nucleic acid sequence of terminator tTEF1.sba"
  Nucleic acid sequence of terminator tTEF1.sba
ggagattgataggacttttctagttgcatatcttttatttttaaatcttatctattagttaattttttgtaatttatccttatatatatagtttggttattctaaaacatcatttcagtatctaaaacctctcttattcattacctttttatttaatggtttttgctacaggcaaaaatttaatggtttttgctacaggcaaaaatcccgccgtggacttattccacgttaactcggttacagggtcatgaaccattttgtcaattatcgaaataacttcttcaaaagtccctcttactt

SEQ ID NO: 96 - DNA, 1113 bp, Saccharomyces cerevisiae
  "nucleic acid sequence of Glutamine synthetase (GLN1)"
  nucleic acid sequence of Glutamine synthetase (GLN1)
atggctgaagcaagcatcgaaaagactcaaattttacaaaaatatctagaactggaccaaagaggtagaataattgccgaatacgtttggatcgatggtactggtaacttacgttccaaaggtagaactttgaagaagagaatcacatccattgaccaattgccagaatggaacttcgacggttcttctaccaaccaagcgccaggccacgactctgacatctatttgaaacccgttgcttactacccagatcccttcaggagaggtgacaacattgttgtcttggccgcatgttacaacaatgacggtactccaaacaagttcaaccacagacacgaagctgccaagctatttgctgctcataaggatgaagaaatctggtttggtctagaacaagaatacactctatttgacatgtatgacgatgtttacggatggccaaagggtgggtacccagctccacaaggtccttactactgtggtgttggtgccggtaaggtttatgccagagacatgatcgaagctcactacagagcttgtttgtatgccggattagaaatttctggtattaacgctgaagtcatgccatctcaatgggaattccaagtcggtccatgtaccggtattgacatgggtgaccaattatggatggccagatactttttgcacagagtggcagaagagtttggtatcaagatctcattccatccaaagccattgaagggtgactggaacggtgccggttgtcacactaacgtttccaccaaggaaatgagacaaccaggtggtatgaaatacatcgaacaagccatcgagaagttatccaagagacacgctgaacacattaagttgtacggtagcgataacgacatgagattaactggtagacatgaaaccgcttccatgactgccttttcttctggtgtcgccaacagaggtagctcaattagaatcccaagatccgtcgccaaggaaggttacggttactttgaagaccgtagaccagcttccaacatcgacccatacttggttacaggtatcatgtgtgaaactgtttgcggtgctattgacaatgctgacatgacgaaggaatttgaaagagaatcttcataa

SEQ ID NO: 97 - protein, 370 aa, Saccharomyces cerevisiae
  "amino acid sequence of Glutamine synthetase (GLN1)"
  amino acid sequence of Glutamine synthetase (GLN1)
MAEASIEKTQILQKYLELDQRGRIIAEYVWIDGTGNLRSKGRTLKKRITSIDQLPEWNFDGSSTNQAPGHDSDIYLKPVAYYPDPFRRGDNIVVLAACYNNDGTPNKFNHRHEAAKLFAAHKDEEIWFGLEQEYTLFDMYDDVYGWPKGGYPAPQGPYYCGVGAGKVYARDMIEAHYRACLYAGLEISGINAEVMPSQWEFQVGPCTGIDMGDQLWMARYFLHRVAEEFGIKISFHPKPLKGDWNGAGCHTNVSTKEMRQPGGMKYIEQAIEKLSKRHAEHIKLYGSDNDMRLTGRHETASMTAFSSGVANRGSSIRIPRSVAKEGYGYFEDRRPASNIDPYLVTGIMCETVCGAIDNADMTKEFERESS

SEQ ID NO: 98 - DNA, 6438 bp, Saccharomyces cerevisiae
  "nucleic acid sequence of Glutamate synthase (GLT1)"
  nucleic acid sequence of Glutamate synthase (GLT1)
atgccagtgttgaaatcagacaatttcgatccattggaagaagcttacgaaggtgggacaattcaaaactataacgatgaacaccatcttcataaatcttgggcaaatgtgattccggacaaacgaggactttacgaccctgattatgaacatgacgcttgtggtgtcggtttcgtagcaaataagcatggtgaacagtctcacaagattgttactgacgctagatatcttttagtgaatatgacacatcgtggtgccgtctcatctgatgggaacggtgacggtgccggtattctgctaggtattcctcacgaatttatgaaaagagaattcaagttagatcttgatctagacatacctgagatgggcaaatacgccgtaggtaacgtcttcttcaagaagaacgaaaaaaataacaagaaaaatttaattaagtgtcagaagattttcgaggatttagctgcatccttcaacttatccgtattaggttggagaaacgtccccgtagattctactattttaggagacgttgcattatctcgtgaacctactattctacagccattattggttccattgtatgatgaaaaacaaccggagtttaatgaaactaaatttagaactcaattgtatcttttaaggaaggaggcctctcttcaaataggactggaaaactggttctatgtttgttccctaaacaataccaccattgtttacaagggtcaattgacgccagctcaagtgtataactactatcccgacttgactaatgcgcatttcaaatcccacatggcgttggtccattcaagattttccactaatactttcccctcttgggatagagctcaacctttacgttggctagctcataatggtgaaattaacaccttaagaggtaacaagaattggatgcgctccagagaaggtgtgatgaattcagcaactttcaaagatgagttagacaaactatacccaattatcgaagaaggtggttctgattcagctgcattggataacgttttagaactattgactattaatggcacattatctctacctgaagctgttatgatgatggttcctgaagcgtatcataaggatatggattctgacctaaaagcatggtacgactgggctgcatgtctgatggaaccttgggatggtccagctttgttaactttcactgatggacgttactgtggtgctatattggatagaaatggtttaagaccttgtcgttattacatcactagtgatgacagagttatctgtgcttcagaggtaggtgtcattcctatcgaaaattcattggttgttcaaaaaggtaaactgaagccaggtgatttattcctagtggatactcaattgggtgaaatggtcgatactaaaaagttaaaatctcaaatctcaaaaagacaagattttaagtcttggttatccaaagtcatcaagttagacgacttgttatcaaaaaccgctaatttggttcctaaagaatttatatcacaggattcattgtctttgaaagttcaaagtgacccacgtctattggccaatggttataccttcgaacaagtcacatttctgttaactccaatggctttaacaggtaaagaagctttaggttcgatgggtaacgatgcgccactggcttgtttaaatgaaaatcctgtcttactttatgattatttcagacaattgtttgctcaagtgaccaatcctccaattgacccaattcgtgaagcaaatgttatgtcgttagaatgttatgtcggacctcaaggcaaccttttggaaatgcattcatctcaatgtgatcgtttattattgaaatctcctattttgcattggaatgagttccaagctttgaaaaacattgaagctgcttacccatcatggtctgtagcagaaattgatatcacattcgacaagagtgagggtctattgggctataccgacacaattgataaaatcactaagttagcgagcgaagcaattgatgatggtaaaaagatcttaataattactgacaggaaaatgggtgccaaccgtgtttccatctcctctttgattgcaatttcatgtattcatcatcacctaatcagaaacaagcagcgttcccaagttgctttgattttggaaacaggtgaagccagagaaattcaccatttctgtgtcctactaggttatggttgtgatggtgtttatccatacttagccatggaaactttggtcagaatgaatagagaaggtctacttcgtaatgtcaacaatgacaatgatacacttgaggaagggcaaatactagaaaattacaagcacgctattgatgcaggtatcttgaaggttatgtctaaaatgggtatctccactctagcatcctacaaaggtgctcaaatttttgaagccctaggtttagataactctattgttgatttgtgtttcacaggtacttcttccagaattagaggtgtaactttcgagtatttggctcaagatgccttttctttacatgagcgtggttatccatccagacaaaccattagtaaatctgttaacttaccagaaagtggtgaataccactttagggatggtggttacaaacacgtcaacgaaccaaccgcaattgcttcgttacaagatactgtcagaaacaaaaatgatgtctcttggcaattatatgtaaagaaggaaatggaagcaattagagactgtacactaagaggactgttagaattagattttgaaaattctgtcagtatccctctagaacaagttgaaccatggactgaaattgccagaagatttgcgtcaggtgcaatgtcttatggttctatttctatggaagctcactctacattggctattgccatgaatcgtttaggggccaaatccaattgtggtgaaggtggtgaagacgcagaacgttctgctgttcaagaaaacggtgatactatgagatctgctatcaaacaagttgcttccgctagattcggtgtaacttcatactacttgtcagatgctgatgaaatccaaattaagattgctcagggtgctaagccgggtgaaggtggtgaactaccagcccacaaagtgtctaaggatatcgcaaaaaccaggcactccacccctaatgttgggttaatctctcctcctcctcatcacgatatttattccattgaagatttgaaacaactgatttatgatttgaaatgtgctaatccaagagcgggaatttctgtaaagttggtttccgaagttggtgttggtattgttgcctctggtgtagctaaggctaaagccgatcatatcttagtttctggtcatgatggtggtacaggtgctgcaagatggacgagtgtcaaatatgcgggtttgccatgggaattaggtctagctgaaactcaccagactttagtcttgaatgatttaagacgtaatgttgttgtccaaaccgatggtcaattgagaactgggtttgatattgctgttgcagttttattaggggcagaatcttttaccttggcaacagttccattaattgctatgggttgtgttatgttaagaagatgtcacttgaactcttgtgctgttggtattgccacacaagatccatatttgagaagtaagtttaagggtcagcccgaacatgttatcaacttcttctattacttgatccaagatttaagacaaatcatggccaagttaggattccgtaccattgacgaaatggtgggtcattctgaaaaattaaagaaaagggacgacgtaaatgccaaagccataaatatcgatttatctcctattttgaccccagcacatgttattcgtccaggtgttccaaccaagttcactaagaaacaagaccacaaactccacacccgtctagataataagttaatcgatgaggctgaagttactttggatcgtggcttaccagtgaatattgacgcctctataatcaatactgatcgtgcactcggttctactttatcttacagagtctcgaagaaatttggtgaagatggtttgccaaaggacaccgttgtcgttaacatagaaggttcagcgggtcaatcttttggtgctttcctagcttctggtatcacttttatcttgaatggtgatgctaatgattatgttggtaaaggtttatccggtggtattattgtcattaaaccaccaaaggattctaaattcaagagtgatgaaaatgtaattgttggtaacacttgtttctatggtgctacttctggtactgcattcatttcaggtagtgccggtgagcgtttcggtgtcagaaactctggtgccaccatcgttgttgagagaattaagggtaacaatgcctttgagtatatgactggtggtcgtgccattgtcttatcacaaatggaatccctaaacgccttctctggtgctactggtggtattgcatactgtttaacttccgattacgacgattttgttggaaagattaacaaagatactgttgagttagaatcattatgtgacccggtcgagattgcgtttgttaagaatttgatccaggagcattggaactacacacaatctgatctagcagccaggattctcggtaatttcaaccattatttgaaagatttcgttaaagtcattccaactgattataagaaagttttgttgaaggagaaagcagaagctgccaaggcaaaggctaaggcaacttcagaatacttaaagaagtttagatcgaaccaagaagttgatgacgaagtcaatactctattgattgctaatcaaaaagctaaagagcaagaaaaaaagaagagtattactatttcaaataaggccactttgaaggagcctaaggttgttgatttagaagatgcagttccagattccaaacagctagagaagaatagcgaaaggattgaaaaaacacgtggttttatgatccacaaacgtcgtcatgagacacacagagatccaagaaccagagttaatgactggaaagaatttactaaccctattaccaagaaggatgccaaatatcaaactgcgagatgtatggattgtggtacaccattctgtttatctgataccggttgtcccctatctaacattatccccaagtttaatgaattgttattcaagaaccaatggaagttggcactggacaaattgctagagacaaacaatttcccagaattcactggaagagtatgtccagcaccctgtgagggagcttgtacactaggtattattgaagacccagtcggcataaaatcggttgaaagaattatcattgacaatgctttcaaggaaggatggattaagccttgtccaccaagtacacgcactggctttacagtgggtgtcattggttctggtccagcaggtttagcgtgtgctgatatgttgaaccgtgccggacatacggtcactgtttatgaaagatccgaccgttgtggtgggttattgatgtatggtattccaaacatgaagttggataaggctatagtgcaacgtcgtattgatctattgagtgccgaaggtattgactttgttaccaacaccgaaattggtaaaaccataagcatggatgagctaaagaacaagcacaatgcagtagtgtatgctatcggttctaccattccacgtgacttacctattaagggtcgtgaattgaagaatattgattttgccatgcagttgttggaatctaacacaaaagctttattgaacaaagatctggaaatcattcgtgaaaagatccaaggtaagaaagtaattgttgtcggtggtggtgacacaggtaacgattgtttaggtacatctgtaagacacggtgcagcatcagttttgaatttcgaattgttgcctgagccaccagtggaacgtgccaaagacaatccatggcctcaatggccgcgtgtcatgagagtggactacggtcatgctgaagtgaaagagcattatggtagagaccctcgtgaatactgcatcttgtccaaggaatttatcggtaacgatgagggtgaagtcactgccatcagaactgtgcgcgtagaatggaagaagtcacaaagtggcgtatggcaaatggtagaaattcccaacagtgaagagatctttgaagccgatatcattttgttgtctatgggtttcgtgggtcctgaattgatcaatggcaacgataacgaagttaagaagacaagacgtggtacgattgccacactcgacgactcctcatactctattgatggaggaaagacttttgcatgtggtgactgtagaagagggcaatctttgattgtctgggccatccaagaaggtagaaaatgtgctgcctctgtcgataagttcctaatggacggcactacgtatctaccaagtaatggtggtatcgttcaacgtgattacaaactattgaaagaattagctagtcaagtctaa

SEQ ID NO: 99 - protein, 2145 aa, Saccharomyces cerevisiae
  "amino acid sequence of Glutamate synthase (GLT1)"
  amino acid sequence of Glutamate synthase (GLT1)
MPVLKSDNFDPLEEAYEGGTIQNYNDEHHLHKSWANVIPDKRGLYDPDYEHDACGVGFVANKHGEQSHKIVTDARYLLVNMTHRGAVSSDGNGDGAGILLGIPHEFMKREFKLDLDLDIPEMGKYAVGNVFFKKNEKNNKKNLIKCQKIFEDLAASFNLSVLGWRNVPVDSTILGDVALSREPTILQPLLVPLYDEKQPEFNETKFRTQLYLLRKEASLQIGLENWFYVCSLNNTTIVYKGQLTPAQVYNYYPDLTNAHFKSHMALVHSRFSTNTFPSWDRAQPLRWLAHNGEINTLRGNKNWMRSREGVMNSATFKDELDKLYPIIEEGGSDSAALDNVLELLTINGTLSLPEAVMMMVPEAYHKDMDSDLKAWYDWAACLMEPWDGPALLTFTDGRYCGAILDRNGLRPCRYYITSDDRVICASEVGVIPIENSLVVQKGKLKPGDLFLVDTQLGEMVDTKKLKSQISKRQDFKSWLSKVIKLDDLLSKTANLVPKEFISQDSLSLKVQSDPRLLANGYTFEQVTFLLTPMALTGKEALGSMGNDAPLACLNENPVLLYDYFRQLFAQVTNPPIDPIREANVMSLECYVGPQGNLLEMHSSQCDRLLLKSPILHWNEFQALKNIEAAYPSWSVAEIDITFDKSEGLLGYTDTIDKITKLASEAIDDGKKILIITDRKMGANRVSISSLIAISCIHHHLIRNKQRSQVALILETGEAREIHHFCVLLGYGCDGVYPYLAMETLVRMNREGLLRNVNNDNDTLEEGQILENYKHAIDAGILKVMSKMGISTLASYKGAQIFEALGLDNSIVDLCFTGTSSRIRGVTFEYLAQDAFSLHERGYPSRQTISKSVNLPESGEYHFRDGGYKHVNEPTAIASLQDTVRNKNDVSWQLYVKKEMEAIRDCTLRGLLELDFENSVSIPLEQVEPWTEIARRFASGAMSYGSISMEAHSTLAIAMNRLGAKSNCGEGGEDAERSAVQENGDTMRSAIKQVASARFGVTSYYLSDADEIQIKIAQGAKPGEGGELPAHKVSKDIAKTRHSTPNVGLISPPPHHDIYSIEDLKQLIYDLKCANPRAGISVKLVSEVGVGIVASGVAKAKADHILVSGHDGGTGAARWTSVKYAGLPWELGLAETHQTLVLNDLRRNVVVQTDGQLRTGFDIAVAVLLGAESFTLATVPLIAMGCVMLRRCHLNSCAVGIATQDPYLRSKFKGQPEHVINFFYYLIQDLRQIMAKLGFRTIDEMVGHSEKLKKRDDVNAKAINIDLSPILTPAHVIRPGVPTKFTKKQDHKLHTRLDNKLIDEAEVTLDRGLPVNIDASIINTDRALGSTLSYRVSKKFGEDGLPKDTVVVNIEGSAGQSFGAFLASGITFILNGDANDYVGKGLSGGIIVIKPPKDSKFKSDENVIVGNTCFYGATSGTAFISGSAGERFGVRNSGATIVVERIKGNNAFEYMTGGRAIVLSQMESLNAFSGATGGIAYCLTSDYDDFVGKINKDTVELESLCDPVEIAFVKNLIQEHWNYTQSDLAARILGNFNHYLKDFVKVIPTDYKKVLLKEKAEAAKAKAKATSEYLKKFRSNQEVDDEVNTLLIANQKAKEQEKKKSITISNKATLKEPKVVDLEDAVPDSKQLEKNSERIEKTRGFMIHKRRHETHRDPRTRVNDWKEFTNPITKKDAKYQTARCMDCGTPFCLSDTGCPLSNIIPKFNELLFKNQWKLALDKLLETNNFPEFTGRVCPAPCEGACTLGIIEDPVGIKSVERIIIDNAFKEGWIKPCPPSTRTGFTVGVIGSGPAGLACADMLNRAGHTVTVYERSDRCGGLLMYGIPNMKLDKAIVQRRIDLLSAEGIDFVTNTEIGKTISMDELKNKHNAVVYAIGSTIPRDLPIKGRELKNIDFAMQLLESNTKALLNKDLEIIREKIQGKKVIVVGGGDTGNDCLGTSVRHGAASVLNFELLPEPPVERAKDNPWPQWPRVMRVDYGHAEVKEHYGRDPREYCILSKEFIGNDEGEVTAIRTVRVEWKKSQSGVWQMVEIPNSEEIFEADIILLSMGFVGPELINGNDNEVKKTRRGTIATLDDSSYSIDGGKTFACGDCRRGQSLIVWAIQEGRKCAASVDKFLMDGTTYLPSNGGIVQRDYKLLKELASQV

SEQ ID NO: 100 - DNA, 300 bp, Saccharomyces cerevisiae
  "nucleic acid sequence of terminator tTDH3"
  nucleic acid sequence of terminator tTDH3
gtgaatttactttaaatcttgcatttaaataaattttctttttatagctttatgacttagtttcaatttatatactattttaatgacattttcgattcattgattgaaagctttgtgttttttcttgatgcgctattgcattgttcttgtctttttcgccacatgtaatatctgtagtagatacctgatacattgtggatgctgagtgaaattttagttaataatggaggcgctcttaataattttggggatattggcttttttttttaaagtttacaaatgaattttttccgccaggat

SEQ ID NO: 101 - DNA, 1788 bp, Artificial Sequence
  "reencoded nucleic acid sequence of hyaluronan synthase (HASA) originating from Chlorella virus CviKI"
  reencoded nucleic acid sequence of hyaluronan synthase (HASA) originating from Chlorella virus CviKI
atgcttttcagttgtttgtccttcgtgatctgccatcttagttttattttgcgttattacaagaggcttctaaaagtgacgatgggaaagaacattataataatggtgagttggtacacaataataacttccaacatcatcgccgtcggtggggcgtctctgattttggccccagccatcactggatacatcttgcactggaacatcgccttgtcaaccatctggggagtttccgcttatgggatattcgtgttcggattcttcctggctcaggttttatttagtgagctaaatcgtaaaagactaagaaagtggatttctctaagaccaaagggttggaacgacgtacgtctggctgtcatcatagctggttacagggaagacccgtacatgtttcagaaatgccttgagtcagtaagggactctgactatggtaatgtcgctcgtcttatctgtgtaattgacggagatgaggacgacgacatgaagatggcagccgtttataaggcgatatataatgacaatatcaagaagccagagtttgtgttatgtgagagcgatgataaggaaggcgagagaattgactcagattttagcagggacatctgcgtcttacaaccacaccgtggcaaaagggagtgcttgtataccggctttcagctggccaaaatggacccgtcggtaaacgccgttgttcttattgactctgacacggtcttggaaaaggacgcaatcttggaagtcgtgtatccattggcctgtgacccggaaattcaagctgtcgcaggagagtgcaaaatatggaacacagatacacttttgtcgttgttggtggcttggagatattattcagccttttgcgtggagagatccgcccaatcattctttaggacagtccagtgtgtaggtggacccttgggcgcctacaagatagatatcatcaaagagatcaaagatccctggatctcccaacgtttcttaggtcagaagtgcacctacggtgacgaccgtaggttaacaaatgaaatcttaatgaggggtaagaaggtcgtcttcactcctttcgcagttggctggagtgactcaccaaccaacgtgttcaggtacatcgtacaacagactaggtggagtaaatcatggtgccgtgagatatggtacactttgtttgctgcgtggaagcacggactaagcggaatttggttggcatttgagtgcctttatcagattacgtacttcttcctagtcatatatttattttcgagactagccgttgaagctgacccaagagcacagaccgcaacagtaatcgtgtctaccacggtagccctgattaagtgtggttacttctcttttcgtgcgaaagatattcgtgctttctacttcgtcctgtacacatttgtctacttcttctgtatgatcccagcaagggtgacagccatgatgacactttgggatatcggctggggcacgcgtggcggaaacgagaaaccaagtgtcggcactagggtcgctctgtgggctaaacagtatttgatagcatacatgtggtgggcagcagttgttggcgctggggtatactccattgttcataattggatgtttgactggaactcactatcctataggttcgcacttgtaggtatatgctcttacatcgtattcatcacaatcgttctagtcatctatttcacaggaaagattaccacatggaatttcaccaaattacagaaggagttaatcaaggatagggtcttatacgatgcttccactaacgcccagactgtataa

SEQ ID NO: 102 - DNA, 1803 bp, Artificial Sequence
  "reencoded nucleic acid sequence of hyaluronan synthase (HASA) originating from Chlorella virus IL-5-2s1"
  reencoded nucleic acid sequence of hyaluronan synthase (HASA) originating from Chlorella virus IL-5-2s1
atggctgcttcattctatgttatcttcttgttcgtaatatgccacctgtccttcgtcttatatcgtcaagttctatacataattttgggtagatactggagtgttaacaagctgacaatgatctcttggtataccattatatcatctaatctaatcgcaatcggtggggcttcccttattttggcaccggccataaccggctacattttgcattggaacatagctctaagcacaatttggggtgtgtcagcctatggcattttcgtgttcgggttctttcttgctcaggttttgttcagtgagcttaacaggaagaggttgagaaaatggatctctttgagaccagataactggaacgcggtgagagttgccgtgataatcgctggttaccgtgaagacccatacatgtttcaaaagtgtttggaatcggtgagagactccgattatggtaacattgcgaggcttatatgcgttatagatggggacgaagatgacgacatgaagatggcagatgtatacaaggctatttacaatgacaatataaagaagccggaaattatcctatgtgagtccgacgacaaagagggagaaaggatagacagtgattttagccgtgatatttgcgtgcttcagcctcacagaggtaagcgtgaatgtttatatactggctttcagttagctaaaatggacccctctgtacacgcggttgtgcttattgactcggatacagttttggagaaggatgccatcctggaagtggtctacccacttgcttgcgaccatgagattcaagcagtcgcaggtgaatgcaagatatggaatacggacaccttattatccatattagtcgcctggcgttactactcagctttctgcgttgagcgtagcgctcagtccttcttccgtactgtgcaatgcgtcggcggtccgttaggggcatacaaaatagacataattaaagagataaaggagccgtggatttcacaaagatttctgggtcagaagtgtacgtacggagatgacagaagattaactaacgaagtgttgatgcgtggaaagaaagtagtcttcacaccttttgcggtaggatggagcgactcgcctactaatgtcttccgttatattgtgcagcagacgaggtggagtaagagctggtgcagggagatttggtatacactgttcgcggcgtggaagcatgggttatcaggcatttggttggcatttgagtgcttgtatcagatcacatacttctttctagtgatatatctgttcagtagactagcagtcgaggctgacccgagagcgcaaactgcaacggttatagtcagcacaatggtttcactaatcaagtgtggatatttctcattccgtgctaaggacattagagcgttttatttcgtactatatacttttgtgtacttcttttgcatgatcccagcaagagtcactgctatgatgaccttgtgggatattgggtggggtactaggggtggaaacgtgaaaccatcgatcggaactaggatctctttgtgggctaagcagtacttaatcgcgtacatgtggtgggcagctgtgatcgccgcaggagtctatagtataatacataattggatgtttgattggaactccttgtcctatcgtttcgcgttaataggcatctgctcgtatatcgtattcattgccattgttatagtgatatacttcacaggtaagatcaccacttggaattttaccaagctacagaaagagttaattgaagatagagtcttgcatgatgccgatgtggacatacagaacgtataa

SEQ ID NO: 103 - DNA, 1686 bp, Artificial Sequence
  "reencoded nucleic acid sequence of hyaluronan synthase (HASA) originating from Chlorella virus CZ-2"
  reencoded nucleic acid sequence of hyaluronan synthase (HASA) originating from Chlorella virus CZ-2
atgacatcttggagaacgattgtgtcagctaaccttttcgcagttggtggggctcttctaatgttagccccagctatcgtgggctatgtatttcagtggaatataggcgtgtccgcagtctggggcatctccgtatacggcgtctttgtgttgggattttatatcgctcaaatcgtcttctctgagttcaacaggatgagattatccgattggataagtcttagaccagacaactggaacgccacaagggttgcggtcattatagctggatacagagaagatccttttatgttcaagaagtgcttagagagtgtgagggattcggaatacggcaacgtagcaaggcttatatgcgtaattgacggagacgaagaagaggacctaaagatggctgagatttacaagcaggtttacaatgacaacgtgaagaaaccaggtgtagtgttatgcgaatcggagaacaagaatggatcgactatagattcggacgtatctaagaatatatgcatactgcaaccccaccgtgggaaacgtgagagcctatataccggtttccaattggcaagcatggacccttccgtacatgcggttgttcttatagattccgacactgtattagagaagaatgctattcttgaggtcgtataccctctatcttgtgaccccaacattaaggccgtcgccggggagtgcaagatatggaatacagacaccatcttgtccatgcttgtctcttggagatacttctctgccttcaatgtcgagcgtggagcccagtcattatggaagactgtgcaatgcgtaggcgggccacttggcgcatacactatcgacatcataaatgaaattaaagacccgtggattacccagacattcctgggcaacaagtgcacttatggcgacgatagacgtcttaccaatgaggttttaatgaggggcaagaagattgtatacactccgtttgccgtcggttggagcgacagtccgacgaatgtcatgaggtacattgtgcagcaaactagatggagtaagtcatggtgcagagagatatggtacacgttaggcagtgcctggaaacatggattctccggcatataccttgcgtttgagtgtatgtaccagataatgtacttcttcttagtcatgtacctgttttcgtatatcgcaataaaggcagacatccgtgctcagactgcaactgtgttggtttctactctagtcaccataataaagagcagttacctagcgctgagggccaagaacctgaaggctttctatttcgttctgtatacctatgtctatttcttttgcatgatacctgctaggattaccgctatgtttacaatgtttgatatagcttggggtacacgtggtggtaatgcgaaaatgacaatcggggctagagtttggctgtgggcgaagcagttcttaataacttatatgtggtgggcaggagtactagcggcgggagtttacagtatagttgacaattggtacttcgattgggctgatatacagtacaggtttgcattggtaggtatttgctcgtatttggtctttgtcagtattgtactggtaatctacttgatcggtaagataacaacgtggaactacacaccgctacagaaggaacttattgaggagagatacttgcataacgcctctgagaatgccccggaagtttaa

SEQ ID NO: 104 - DNA, 1677 bp, Artificial Sequence
  "reencoded nucleic acid sequence of hyaluronan synthase (HASA) originating from Chlorella virus CVG-1"
  reencoded nucleic acid sequence of hyaluronan synthase (HASA) originating from Chlorella virus CVG-1
atgacttcttggcgtacaattgtttctgctaacttgttcgcagttggtggcgccttgttgatgttagctcccgcgatagccggttatgtatttaaatggaacataggcgtttctgccgtttggggtatttcagtgtacggggtcttcgtgcttggtttctatattgcacaggtagtcttcagcgagtttaataggatgcagctgtcagactggatctcattgagacccgacaactggaacgccaccagagtagcggtaattattgctggttacagggaagacccctttatgttcaagaagtgcctagaatctgtgagagactcagaatacgggaacatagcgaggctaatctgtgttatcgacggcgatgaagaggaagaccttaagatggctgagatatacaagcaagtatacaacgacaacgtcaagacccccggtgttgtgctatgcgagaatgaaaataagaatggtagcaccattgacccagattttagtaagaacatctgcattctgcaaccacacaggggcaaacgtgaatctttgtacaccggattccagatggctggcatggacccatcagtgcacgcagttgtacttatagacagtgatactgttcttgaaaagaacgctatcctagaggttgtgtaccctctatcttgtgatccaaatatcaaagctgtcgcgggagagtgtaaaatctggaacacagataccattttgtctatgctagtttcatggcgttatttctcggctttcaacgtggagagaggcgcacagtccctttggaaaacagtccagtgtgtcggcgggcctttgggagcatacactatagacatcataaacgagataaaagacccctggattactcagacattcttaggaaacaaatgtacgtatggtgacgacagaaggttaaccaatgaagtgcttatgaggggaaagaagattgtctatactccctttgctgtcggttggtccgattcgcccacaaacgttatgaggtacatcgtccagcagacaaggtggtctaagagctggtgccgtgagatttggtacaccttgggatcagcatggaaacatggtttctccggaatctacttagcgttcgagtgcatgtaccagattatgtatttctttattgtgatgtatttgttcagttacattgccattaaagccaacatcagggcacaagcagccacggtattggtcagtacgcttgtcgcagtaatcaaatctagttatttggcattaagagcgaagaacctaaaagctttgtatttcgtcctgtatacctacgtctacttcttctgcatgattccagctagaataacagcgatgttcacgatgttcgatattgcatggggtactagaggcggtaacgcaaagatgacgatcggtgctagagtctggttgtgggctaaacaattcttaattacatacatgtggtgggtgggagttttggccgctggggtctacagtatagtcgataactggtacttcgactgggcggacatccagtacagattcgcgctagtggggatttgcagttacttaggtttcgtttccataatgctggtattctatctgattggtaaaataactacgtggaattacactcctctacaaaaggagctgattaaagagaggttacacgccgctaatgcaacagaggtctaa

SEQ ID NO: 105 - protein, 595 aa, Artificial Sequence
  "amino acid sequence of hyaluronan synthase (HASA) originating from Chlorella virus CviKI"
  amino acid sequence of hyaluronan synthase (HASA) originating from Chlorella virus CviKI
MLFSCLSFVICHLSFILRYYKRLLKVTMGKNIIIMVSWYTIITSNIIAVGGASLILAPAITGYILHWNIALSTIWGVSAYGIFVFGFFLAQVLFSELNRKRLRKWISLRPKGWNDVRLAVIIAGYREDPYMFQKCLESVRDSDYGNVARLICVIDGDEDDDMKMAAVYKAIYNDNIKKPEFVLCESDDKEGERIDSDFSRDICVLQPHRGKRECLYTGFQLAKMDPSVNAVVLIDSDTVLEKDAILEVVYPLACDPEIQAVAGECKIWNTDTLLSLLVAWRYYSAFCVERSAQSFFRTVQCVGGPLGAYKIDIIKEIKDPWISQRFLGQKCTYGDDRRLTNEILMRGKKVVFTPFAVGWSDSPTNVFRYIVQQTRWSKSWCREIWYTLFAAWKHGLSGIWLAFECLYQITYFFLVIYLFSRLAVEADPRAQTATVIVSTTVALIKCGYFSFRAKDIRAFYFVLYTFVYFFCMIPARVTAMMTLWDIGWGTRGGNEKPSVGTRVALWAKQYLIAYMWWAAVVGAGVYSIVHNWMFDWNSLSYRFALVGICSYIVFITIVLVIYFTGKITTWNFTKLQKELIKDRVLYDASTNAQTV

SEQ ID NO: 106 - protein, 600 aa, Artificial Sequence
  "amino acid sequence of hyaluronan synthase (HASA) originating from Chlorella virus IL-5-2s1"
  amino acid sequence of hyaluronan synthase (HASA) originating from Chlorella virus IL-5-2s1
MAASFYVIFLFVICHLSFVLYRQVLYIILGRYWSVNKLTMISWYTIISSNLIAIGGASLILAPAITGYILHWNIALSTIWGVSAYGIFVFGFFLAQVLFSELNRKRLRKWISLRPDNWNAVRVAVIIAGYREDPYMFQKCLESVRDSDYGNIARLICVIDGDEDDDMKMADVYKAIYNDNIKKPEIILCESDDKEGERIDSDFSRDICVLQPHRGKRECLYTGFQLAKMDPSVHAVVLIDSDTVLEKDAILEVVYPLACDHEIQAVAGECKIWNTDTLLSILVAWRYYSAFCVERSAQSFFRTVQCVGGPLGAYKIDIIKEIKEPWISQRFLGQKCTYGDDRRLTNEVLMRGKKVVFTPFAVGWSDSPTNVFRYIVQQTRWSKSWCREIWYTLFAAWKHGLSGIWLAFECLYQITYFFLVIYLFSRLAVEADPRAQTATVIVSTMVSLIKCGYFSFRAKDIRAFYFVLYTFVYFFCMIPARVTAMMTLWDIGWGTRGGNVKPSIGTRISLWAKQYLIAYMWWAAVIAAGVYSIIHNWMFDWNSLSYRFALIGICSYIVFIAIVIVIYFTGKITTWNFTKLQKELIEDRVLHDADVDIQNV

SEQ ID NO: 107 - protein, 561 aa, Artificial Sequence
  "amino acid sequence of hyaluronan synthase (HASA) originating from Chlorella virus CZ-2"
  amino acid sequence of hyaluronan synthase (HASA) originating from Chlorella virus CZ-2
MTSWRTIVSANLFAVGGALLMLAPAIVGYVFQWNIGVSAVWGISVYGVFVLGFYIAQIVFSEFNRMRLSDWISLRPDNWNATRVAVIIAGYREDPFMFKKCLESVRDSEYGNVARLICVIDGDEEEDLKMAEIYKQVYNDNVKKPGVVLCESENKNGSTIDSDVSKNICILQPHRGKRESLYTGFQLASMDPSVHAVVLIDSDTVLEKNAILEVVYPLSCDPNIKAVAGECKIWNTDTILSMLVSWRYFSAFNVERGAQSLWKTVQCVGGPLGAYTIDIINEIKDPWITQTFLGNKCTYGDDRRLTNEVLMRGKKIVYTPFAVGWSDSPTNVMRYIVQQTRWSKSWCREIWYTLGSAWKHGFSGIYLAFECMYQIMYFFLVMYLFSYIAIKADIRAQTATVLVSTLVTIIKSSYLALRAKNLKAFYFVLYTYVYFFCMIPARITAMFTMFDIAWGTRGGNAKMTIGARVWLWAKQFLITYMWWAGVLAAGVYSIVDNWYFDWADIQYRFALVGICSYLVFVSIVLVIYLIGKITTWNYTPLQKELIEERYLHNASENAPEV

SEQ ID NO: 108 - protein, 558 aa, Artificial Sequence
  "amino acid sequence of hyaluronan synthase (HASA) originating from Chlorella virus CVG-1"
  amino acid sequence of hyaluronan synthase (HASA) originating from Chlorella virus CVG-1
MTSWRTIVSANLFAVGGALLMLAPAIAGYVFKWNIGVSAVWGISVYGVFVLGFYIAQVVFSEFNRMQLSDWISLRPDNWNATRVAVIIAGYREDPFMFKKCLESVRDSEYGNIARLICVIDGDEEEDLKMAEIYKQVYNDNVKTPGVVLCENENKNGSTIDPDFSKNICILQPHRGKRESLYTGFQMAGMDPSVHAVVLIDSDTVLEKNAILEVVYPLSCDPNIKAVAGECKIWNTDTILSMLVSWRYFSAFNVERGAQSLWKTVQCVGGPLGAYTIDIINEIKDPWITQTFLGNKCTYGDDRRLTNEVLMRGKKIVYTPFAVGWSDSPTNVMRYIVQQTRWSKSWCREIWYTLGSAWKHGFSGIYLAFECMYQIMYFFIVMYLFSYIAIKANIRAQAATVLVSTLVAVIKSSYLALRAKNLKALYFVLYTYVYFFCMIPARITAMFTMFDIAWGTRGGNAKMTIGARVWLWAKQFLITYMWWVGVLAAGVYSIVDNWYFDWADIQYRFALVGICSYLGFVSIMLVFYLIGKITTWNYTPLQKELIKERLHAANATEV